European Patent Specification EP 3 697 426 B1, published July 26, 2023. Title: COMPOSITIONS AND METHODS FOR TREATING CANCER WITH ANTI-CD22 IMMUNOTHERAPY. Applicant: LENTIGEN TECHNOLOGY, INC THE DEPARTMENT OF HEALTH AND HUMAN SERVICES, UNITED STATES OF AMERICA. The sequence listing filed with the application follows.

SEQUENCE LISTING (206 sequences)

SEQ ID NO: 1 - DNA, 732 bp, Artificial Sequence
  Description of Artificial Sequence: Synthetic polynucleotide
caagtacaactccagcaaagcgggcctggtctggtgaagccgtcacagacgctttcacttacgtgtgcgatctccggtgactccgtgagttctaatagcgcggcttggaactggattaggcagtctccatcccgaggattggaatggctcggcaggacttattatagaagtaagtggtacaacgattatgcagtctctgtgaaatctcgcatcaccattaacccagacacgtctaagaatcagttcagtcttcaactcaactctgtaacccccgaagatacagcggtctactactgtgctcaggaggtgcaaccccacgatgcttttgatatctggggccagggtaccatggttacggtgtcttctgggggaggggggtccggtgggggaggatcagggggtgggggcagcgacatacaaatgacgcaatccccgtcttctgtttctgcgtctgtcggagataaagtaacaataacctgtcgagcgtcacaggacgttagtggctggcttgcgtggtatcagcaaaaaccggggctcgccccgcaattgcttatatttggagcgagtactcttcagggcgaggtacctagcagattttctgggtccggctcaggtacggacttcaccctgaccatatctagcttgcagcctgaagatttcgccacctactattgtcaacaggcgaagaactttccatatacgttcgggcagggtacgaaattggagataaaa

SEQ ID NO: 2 - protein, 245 aa, Artificial Sequence
  Description of Artificial Sequence: Synthetic polypeptide
QVQLQQSGPGLVKPSQTLSLTCAISGDSVSSNSAAWNWIRQSPSRGLEWLGRTYYRSKWYNDYAVSVKSRITINPDTSKNQFSLQLNSVTPEDTAVYYCAQEVQPHDAFDIWGQGTMVTVSSGGGGSGGGGSGGGGSDIQMTQSPSSVSASVGDKVTITCRASQDVSGWLAWYQQKPGLAPQLLIFGASTLQGEVPSRFSGSGSGTDFTLTISSLQPEDFATYYCQQAKNFPYTFGQGTKLEIKR

SEQ ID NO: 3 - DNA, 1476 bp, Artificial Sequence
  Description of Artificial Sequence: Synthetic polynucleotide
atgcttctcctggtgacaagccttctgctctgtgagttaccacacccagcattcctcctgatcccacaagtacaactccagcaaagcgggcctggtctggtgaagccgtcacagacgctttcacttacgtgtgcgatctccggtgactccgtgagttctaatagcgcggcttggaactggattaggcagtctccatcccgaggattggaatggctcggcaggacttattatagaagtaagtggtacaacgattatgcagtctctgtgaaatctcgcatcaccattaacccagacacgtctaagaatcagttcagtcttcaactcaactctgtaacccccgaagatacagcggtctactactgtgctcaggaggtgcaaccccacgatgcttttgatatctggggccagggtaccatggttacggtgtcttctgggggaggggggtccggtgggggaggatcagggggtgggggcagcgacatacaaatgacgcaatccccgtcttctgtttctgcgtctgtcggagataaagtaacaataacctgtcgagcgtcacaggacgttagtggctggcttgcgtggtatcagcaaaaaccggggctcgccccgcaattgcttatatttggagcgagtactcttcagggcgaggtacctagcagattttctgggtccggctcaggtacggacttcaccctgaccatatctagcttgcagcctgaagatttcgccacctactattgtcaacaggcgaagaactttccatatacgttcgggcagggtacgaaattggagataaaagcggccgcaactaccacccctgcccctcggccgccgactccggccccaaccatcgcaagccaacccctctccttgcgccccgaagcttgccgcccggccgcgggtggagccgtgcatacccgggggctggactttgcctgcgatatctacatttgggccccgctggccggcacttgcggcgtgctcctgctgtcgctggtcatcaccctttactgcaagaggggccggaagaagctgctttacatcttcaagcagccgttcatgcggcccgtgcagacgactcaggaagaggacggatgctcgtgcagattccctgaggaggaagaggggggatgcgaactgcgcgtcaagttctcacggtccgccgacgcccccgcatatcaacagggccagaatcagctctacaacgagctgaacctgggaaggagagaggagtacgacgtgctggacaagcgacgcggacgcgacccggagatgggggggaaaccacggcggaaaaaccctcaggaaggactgtacaacgaactccagaaagacaagatggcggaagcctactcagaaatcgggatgaagggagagcggaggaggggaaagggtcacgacgggctgtaccagggactgagcaccgccactaaggatacctacgatgccttgcatatgcaagcactcccaccccgg

SEQ ID NO: 4 - protein, 492 aa, Artificial Sequence
  Description of Artificial Sequence: Synthetic polypeptide
MLLLVTSLLLCELPHPAFLLIPQVQLQQSGPGLVKPSQTLSLTCAISGDSVSSNSAAWNWIRQSPSRGLEWLGRTYYRSKWYNDYAVSVKSRITINPDTSKNQFSLQLNSVTPEDTAVYYCAQEVQPHDAFDIWGQGTMVTVSSGGGGSGGGGSGGGGSDIQMTQSPSSVSASVGDKVTITCRASQDVSGWLAWYQQKPGLAPQLLIFGASTLQGEVPSRFSGSGSGTDFTLTISSLQPEDFATYYCQQAKNFPYTFGQGTKLEIKAAATTTPAPRPPTPAPTIASQPLSLRPEACRPAAGGAVHTRGLDFACDIYIWAPLAGTCGVLLLSLVITLYCKRGRKKLLYIFKQPFMRPVQTTQEEDGCSCRFPEEEEGGCELRVKFSRSADAPAYQQGQNQLYNELNLGRREEYDVLDKRRGRDPEMGGKPRRKNPQEGLYNELQKDKMAEAYSEIGMKGERRRGKGHDGLYQGLSTATKDTYDALHMQALPPR

SEQ ID NO: 5 - protein, 6 aa, Artificial Sequence
  Description of Artificial Sequence: Synthetic peptide
QDVSGW

SEQ ID NO: 6 - protein, 3 aa, Artificial Sequence
  Description of Artificial Sequence: Synthetic peptide
GAS

SEQ ID NO: 7 - protein, 9 aa, Artificial Sequence
  Description of Artificial Sequence: Synthetic peptide
QQAKNFPYT

SEQ ID NO: 8 - protein, 10 aa, Artificial Sequence
  Description of Artificial Sequence: Synthetic peptide
GDSVSSNSAA

SEQ ID NO: 9 - protein, 9 aa, Artificial Sequence
  Description of Artificial Sequence: Synthetic peptide
TYYRSKWYN

SEQ ID NO: 10 - protein, 12 aa, Artificial Sequence
  Description of Artificial Sequence: Synthetic peptide
AQEVQPHDAFDI

SEQ ID NO: 11 - DNA, 732 bp, Artificial Sequence
  Description of Artificial Sequence: Synthetic polynucleotide
caagtacagctgcaacaatctggccctgggcttgtgaaaccctctcagactttgtccttgacgtgcgcgataagtggcgattcagttagttctaacagcgccgcttggaactggattagacagagccccagtcggggactcgaatggcttggccggacttattatcgcagtaaatggtataatgattatgctgtgagtgtgaaaagtaggatcacaatcaaccccgatacgagcaagaatcaattctcattgcaactgaacagcgtcactcccgaggatacagctgtatattattgtgcaagagaaggtgggtggtatggcgagatggatgtatgggggaaaggaactacggtaactgtgtccagtggcggaggcggttcaggtggtggaggctctggaggaggagggtccgaaatcgtgcttacccagtctccggctactctgagcgttagtccgggtgaaagggcctcactctcttgtcgagcttcacagtcagtctcttcctacttggcttggtatcagcagaagccaggtcaggcgccccgcttgctcatttacgacgcaagcacacgagcgacaggcattccagacagattttctggttctggttctggcacggactttactcttactataaactcacttgaggcagaggatgctgcgacttactattgtcaccaatcaagctctctgccttacacctttgggcaaggcaccaaactcgaaatcaag

SEQ ID NO: 12 - protein, 245 aa, Artificial Sequence
  Description of Artificial Sequence: Synthetic polypeptide
QVQLQQSGPGLVKPSQTLSLTCAISGDSVSSNSAAWNWIRQSPSRGLEWLGRTYYRSKWYNDYAVSVKSRITINPDTSKNQFSLQLNSVTPEDTAVYYCAREGGWYGEMDVWGKGTTVTVSSGGGGSGGGGSGGGGSEIVLTQSPATLSVSPGERASLSCRASQSVSSYLAWYQQKPGQAPRLLIYDASTRATGIPDRFSGSGSGTDFTLTINSLEAEDAATYYCHQSSSLPYTFGQGTKLEIKR

SEQ ID NO: 13 - DNA, 1491 bp, Artificial Sequence
  Description of Artificial Sequence: Synthetic polynucleotide
atgctgctgttggtgacatcacttctgctctgtgaactcccccatccagcctttctgcttataccgcaagtacagctgcaacaatctggccctgggcttgtgaaaccctctcagactttgtccttgacgtgcgcgataagtggcgattcagttagttctaacagcgccgcttggaactggattagacagagccccagtcggggactcgaatggcttggccggacttattatcgcagtaaatggtataatgattatgctgtgagtgtgaaaagtaggatcacaatcaaccccgatacgagcaagaatcaattctcattgcaactgaacagcgtcactcccgaggatacagctgtatattattgtgcaagagaaggtgggtggtatggcgagatggatgtatgggggaaaggaactacggtaactgtgtccagtggcggaggcggttcaggtggtggaggctctggaggaggagggtccgaaatcgtgcttacccagtctccggctactctgagcgttagtccgggtgaaagggcctcactctcttgtcgagcttcacagtcagtctcttcctacttggcttggtatcagcagaagccaggtcaggcgccccgcttgctcatttacgacgcaagcacacgagcgacaggcattccagacagattttctggttctggttctggcacggactttactcttactataaactcacttgaggcagaggatgctgcgacttactattgtcaccaatcaagctctctgccttacacctttgggcaaggcaccaaactcgaaatcaaggttacggtatcatctgcggccgcaactaccacccctgcccctcggccgccgactccggccccaaccatcgcaagccaacccctctccttgcgccccgaagcttgccgcccggccgcgggtggagccgtgcatacccgggggctggactttgcctgcgatatctacatttgggccccgctggccggcacttgcggcgtgctcctgctgtcgctggtcatcaccctttactgcaagaggggccggaagaagctgctttacatcttcaagcagccgttcatgcggcccgtgcagacgactcaggaagaggacggatgctcgtgcagattccctgaggaggaagaggggggatgcgaactgcgcgtcaagttctcacggtccgccgacgcccccgcatatcaacagggccagaatcagctctacaacgagctgaacctgggaaggagagaggagtacgacgtgctggacaagcgacgcggacgcgacccggagatgggggggaaaccacggcggaaaaaccctcaggaaggactgtacaacgaactccagaaagacaagatggcggaagcctactcagaaatcgggatgaagggagagcggaggaggggaaagggtcacgacgggctgtaccagggactgagcaccgccactaaggatacctacgatgccttgcatatgcaagcactcccaccccgg

SEQ ID NO: 14 - protein, 497 aa, Artificial Sequence
  Description of Artificial Sequence: Synthetic polypeptide
MLLLVTSLLLCELPHPAFLLIPQVQLQQSGPGLVKPSQTLSLTCAISGDSVSSNSAAWNWIRQSPSRGLEWLGRTYYRSKWYNDYAVSVKSRITINPDTSKNQFSLQLNSVTPEDTAVYYCAREGGWYGEMDVWGKGTTVTVSSGGGGSGGGGSGGGGSEIVLTQSPATLSVSPGERASLSCRASQSVSSYLAWYQQKPGQAPRLLIYDASTRATGIPDRFSGSGSGTDFTLTINSLEAEDAATYYCHQSSSLPYTFGQGTKLEIKVTVSSAAATTTPAPRPPTPAPTIASQPLSLRPEACRPAAGGAVHTRGLDFACDIYIWAPLAGTCGVLLLSLVITLYCKRGRKKLLYIFKQPFMRPVQTTQEEDGCSCRFPEEEEGGCELRVKFSRSADAPAYQQGQNQLYNELNLGRREEYDVLDKRRGRDPEMGGKPRRKNPQEGLYNELQKDKMAEAYSEIGMKGERRRGKGHDGLYQGLSTATKDTYDALHMQALPPR

SEQ ID NO: 15 - protein, 6 aa, Artificial Sequence
  Description of Artificial Sequence: Synthetic peptide
QSVSSY

SEQ ID NO: 16 - protein, 3 aa, Artificial Sequence
  Description of Artificial Sequence: Synthetic peptide
DAS

SEQ ID NO: 17 - protein, 9 aa, Artificial Sequence
  Description of Artificial Sequence: Synthetic peptide
HQSSSLPYT

SEQ ID NO: 18 - protein, 10 aa, Artificial Sequence
  Description of Artificial Sequence: Synthetic peptide
GDSVSSNSAA

SEQ ID NO: 19 - protein, 9 aa, Artificial Sequence
  Description of Artificial Sequence: Synthetic peptide
TYYRSKWYN

SEQ ID NO: 20 - protein, 12 aa, Artificial Sequence
  Description of Artificial Sequence: Synthetic peptide
AREGGWYGEMDV

SEQ ID NO: 21 - DNA, 744 bp, Artificial Sequence
  Description of Artificial Sequence: Synthetic polynucleotide
caagtacagctccaacagagtggacctggtctcgttaagccgtcccaaacactgtctttgacgtgcgctattagtggcgacagcgtatcatccaattctgctgcttggaactggattagacagtcaccgtccagaggcttggaatggctgggcaggacgtactaccgctcaaaatggtataacgattacgcggttagtgtcaaatccaggattaccattaaccctgacacaagtaagaatcagttttctcttcagctgaattccctgactcctgaggatacggccgtttactactgtgcccgagaacaccagaatgaggcggcttttgatatttgggggcaaggaacaatggtcacagttagcagtggggggggtggctccgggggaggtggttccggcggcggtggttctcaatccgtcctgacacaacctccctcagcgagcgggactcccggtcaaagggtgaccatctcttgttctgggggaggtagtaacatcgggacaaatactgcgtcctggtatcagcaactccctgggaccgctcccaagttgttgatatatcgcaatacgcaacgacctagtgggatacctgatagattcagcggaagcaaaagtggtacgagtgcgtctttggcaatatctggcctccagtccgaggacgaagcggattactattgtgcggcctgggatgactcactgaatggttatgtgttcggtgcaggtactcaactcaccgtacttggt

SEQ ID NO: 22 - protein, 248 aa, Artificial Sequence
  Description of Artificial Sequence: Synthetic polypeptide
QVQLQQSGPGLVKPSQTLSLTCAISGDSVSSNSAAWNWIRQSPSRGLEWLGRTYYRSKWYNDYAVSVKSRITINPDTSKNQFSLQLNSLTPEDTAVYYCAREHQNEAAFDIWGQGTMVTVSSGGGGSGGGGSGGGGSQSVLTQPPSASGTPGQRVTISCSGGGSNIGTNTASWYQQLPGTAPKLLIYRNTQRPSGIPDRFSGSKSGTSASLAISGLQSEDEADYYCAAWDDSLNGYVFGAGTQLTVLG

SEQ ID NO: 23 - DNA, 1488 bp, Artificial Sequence
  Description of Artificial Sequence: Synthetic polynucleotide
atgcttctcctggtgacaagccttctgctctgtgagttaccacacccagcattcctcctgatcccacaagtacagctccaacagagtggacctggtctcgttaagccgtcccaaacactgtctttgacgtgcgctattagtggcgacagcgtatcatccaattctgctgcttggaactggattagacagtcaccgtccagaggcttggaatggctgggcaggacgtactaccgctcaaaatggtataacgattacgcggttagtgtcaaatccaggattaccattaaccctgacacaagtaagaatcagttttctcttcagctgaattccctgactcctgaggatacggccgtttactactgtgcccgagaacaccagaatgaggcggcttttgatatttgggggcaaggaacaatggtcacagttagcagtggggggggtggctccgggggaggtggttccggcggcggtggttctcaatccgtcctgacacaacctccctcagcgagcgggactcccggtcaaagggtgaccatctcttgttctgggggaggtagtaacatcgggacaaatactgcgtcctggtatcagcaactccctgggaccgctcccaagttgttgatatatcgcaatacgcaacgacctagtgggatacctgatagattcagcggaagcaaaagtggtacgagtgcgtctttggcaatatctggcctccagtccgaggacgaagcggattactattgtgcggcctgggatgactcactgaatggttatgtgttcggtgcaggtactcaactcaccgtacttggtgcggccgcaactaccacccctgcccctcggccgccgactccggccccaaccatcgcaagccaacccctctccttgcgccccgaagcttgccgcccggccgcgggtggagccgtgcatacccgggggctggactttgcctgcgatatctacatttgggccccgctggccggcacttgcggcgtgctcctgctgtcgctggtcatcaccctttactgcaagaggggccggaagaagctgctttacatcttcaagcagccgttcatgcggcccgtgcagacgactcaggaagaggacggatgctcgtgcagattccctgaggaggaagaggggggatgcgaactgcgcgtcaagttctcacggtccgccgacgcccccgcatatcaacagggccagaatcagctctacaacgagctgaacctgggaaggagagaggagtacgacgtgctggacaagcgacgcggacgcgacccggagatgggggggaaaccacggcggaaaaaccctcaggaaggactgtacaacgaactccagaaagacaagatggcggaagcctactcagaaatcgggatgaagggagagcggaggaggggaaagggtcacgacgggctgtaccagggactgagcaccgccactaaggatacctacgatgccttgcatatgcaagcactcccaccccgg

SEQ ID NO: 24 - protein, 496 aa, Artificial Sequence
  Description of Artificial Sequence: Synthetic polypeptide
MLLLVTSLLLCELPHPAFLLIPQVQLQQSGPGLVKPSQTLSLTCAISGDSVSSNSAAWNWIRQSPSRGLEWLGRTYYRSKWYNDYAVSVKSRITINPDTSKNQFSLQLNSLTPEDTAVYYCAREHQNEAAFDIWGQGTMVTVSSGGGGSGGGGSGGGGSQSVLTQPPSASGTPGQRVTISCSGGGSNIGTNTASWYQQLPGTAPKLLIYRNTQRPSGIPDRFSGSKSGTSASLAISGLQSEDEADYYCAAWDDSLNGYVFGAGTQLTVLGAAATTTPAPRPPTPAPTIASQPLSLRPEACRPAAGGAVHTRGLDFACDIYIWAPLAGTCGVLLLSLVITLYCKRGRKKLLYIFKQPFMRPVQTTQEEDGCSCRFPEEEEGGCELRVKFSRSADAPAYQQGQNQLYNELNLGRREEYDVLDKRRGRDPEMGGKPRRKNPQEGLYNELQKDKMAEAYSEIGMKGERRRGKGHDGLYQGLSTATKDTYDALHMQALPPR

SEQ ID NO: 25 - protein, 8 aa, Artificial Sequence
  Description of Artificial Sequence: Synthetic peptide
GSNIGTNT

SEQ ID NO: 26 - protein, 3 aa, Artificial Sequence
  Description of Artificial Sequence: Synthetic peptide
RNT

SEQ ID NO: 27 - protein, 11 aa, Artificial Sequence
  Description of Artificial Sequence: Synthetic peptide
AAWDDSLNGYV

SEQ ID NO: 28 - protein, 10 aa, Artificial Sequence
  Description of Artificial Sequence: Synthetic peptide
GDSVSSNSAA

SEQ ID NO: 29 - protein, 9 aa, Artificial Sequence
  Description of Artificial Sequence: Synthetic peptide
TYYRSKWYN

SEQ ID NO: 30 - protein, 12 aa, Artificial Sequence
  Description of Artificial Sequence: Synthetic peptide
AREHQNEAAFDI

SEQ ID NO: 31 - DNA, 729 bp, Artificial Sequence
  Description of Artificial Sequence: Synthetic polynucleotide
caagtccagttgcaacagtccgggccaggtctggttaagccatcccaaactctgagtttgacgtgcgctattagcggagattccgtgtccagcaattctgcaacctggaattggatccggcagagtccgagtggcggtttggaatggctcggacgcacttactacaggagcaaatggtacgatgattatgctgtttctgtgcgctctcgaatcaccatgaatcctgatacttctaagaaccaattttctttgcagttgaactccgtcacgcctgaagatactgcggtctactattgcgcacgcgaaggcgtagccggcgattttgattactgggggcaaggaacattggtcacggtctcctctggtggaggaggatcaggaggcgggggttcaggtggaggtgggagcgatattcaacttacgcagtctccgagcagtctttctgcttccgtgggagaccgagtgacgattacttgtagggcatctcagtcaataagttcctatcttaactggtatcagcagaagcctggaaaggctccaaaacttcttatttatgccgcatcctcattgcaatccggcgtgccttcccgattttccggatctggctcaggcactgactttaccttgactattagttcccttcaaccagaagattttgctacctattactgccaacaatcatacagtaccccatatacattcggccaaggcacgaaattggagattaaa

SEQ ID NO: 32 - protein, 244 aa, Artificial Sequence
  Description of Artificial Sequence: Synthetic polypeptide
QVQLQQSGPGLVKPSQTLSLTCAISGDSVSSNSATWNWIRQSPSGGLEWLGRTYYRSKWYDDYAVSVRSRITMNPDTSKNQFSLQLNSVTPEDTAVYYCAREGVAGDFDYWGQGTLVTVSSGGGGSGGGGSGGGGSDIQLTQSPSSLSASVGDRVTITCRASQSISSYLNWYQQKPGKAPKLLIYAASSLQSGVPSRFSGSGSGTDFTLTISSLQPEDFATYYCQQSYSTPYTFGQGTKLEIKR

SEQ ID NO: 33 - DNA, 1473 bp, Artificial Sequence
  Description of Artificial Sequence: Synthetic polynucleotide
atgcttctcctggtgacaagccttctgctctgtgagttaccacacccagcattcctcctgatcccacaagtccagttgcaacagtccgggccaggtctggttaagccatcccaaactctgagtttgacgtgcgctattagcggagattccgtgtccagcaattctgcaacctggaattggatccggcagagtccgagtggcggtttggaatggctcggacgcacttactacaggagcaaatggtacgatgattatgctgtttctgtgcgctctcgaatcaccatgaatcctgatacttctaagaaccaattttctttgcagttgaactccgtcacgcctgaagatactgcggtctactattgcgcacgcgaaggcgtagccggcgattttgattactgggggcaaggaacattggtcacggtctcctctggtggaggaggatcaggaggcgggggttcaggtggaggtgggagcgatattcaacttacgcagtctccgagcagtctttctgcttccgtgggagaccgagtgacgattacttgtagggcatctcagtcaataagttcctatcttaactggtatcagcagaagcctggaaaggctccaaaacttcttatttatgccgcatcctcattgcaatccggcgtgccttcccgattttccggatctggctcaggcactgactttaccttgactattagttcccttcaaccagaagattttgctacctattactgccaacaatcatacagtaccccatatacattcggccaaggcacgaaattggagattaaagcggccgcaactaccacccctgcccctcggccgccgactccggccccaaccatcgcaagccaacccctctccttgcgccccgaagcttgccgcccggccgcgggtggagccgtgcatacccgggggctggactttgcctgcgatatctacatttgggccccgctggccggcacttgcggcgtgctcctgctgtcgctggtcatcaccctttactgcaagaggggccggaagaagctgctttacatcttcaagcagccgttcatgcggcccgtgcagacgactcaggaagaggacggatgctcgtgcagattccctgaggaggaagaggggggatgcgaactgcgcgtcaagttctcacggtccgccgacgcccccgcatatcaacagggccagaatcagctctacaacgagctgaacctgggaaggagagaggagtacgacgtgctggacaagcgacgcggacgcgacccggagatgggggggaaaccacggcggaaaaaccctcaggaaggactgtacaacgaactccagaaagacaagatggcggaagcctactcagaaatcgggatgaagggagagcggaggaggggaaagggtcacgacgggctgtaccagggactgagcaccgccactaaggatacctacgatgccttgcatatgcaagcactcccaccccgg

SEQ ID NO: 34 - protein, 491 aa, Artificial Sequence
  Description of Artificial Sequence: Synthetic polypeptide
MLLLVTSLLLCELPHPAFLLIPQVQLQQSGPGLVKPSQTLSLTCAISGDSVSSNSATWNWIRQSPSGGLEWLGRTYYRSKWYDDYAVSVRSRITMNPDTSKNQFSLQLNSVTPEDTAVYYCAREGVAGDFDYWGQGTLVTVSSGGGGSGGGGSGGGGSDIQLTQSPSSLSASVGDRVTITCRASQSISSYLNWYQQKPGKAPKLLIYAASSLQSGVPSRFSGSGSGTDFTLTISSLQPEDFATYYCQQSYSTPYTFGQGTKLEIKAAATTTPAPRPPTPAPTIASQPLSLRPEACRPAAGGAVHTRGLDFACDIYIWAPLAGTCGVLLLSLVITLYCKRGRKKLLYIFKQPFMRPVQTTQEEDGCSCRFPEEEEGGCELRVKFSRSADAPAYQQGQNQLYNELNLGRREEYDVLDKRRGRDPEMGGKPRRKNPQEGLYNELQKDKMAEAYSEIGMKGERRRGKGHDGLYQGLSTATKDTYDALHMQALPPR

SEQ ID NO: 35 - protein, 6 aa, Artificial Sequence
  Description of Artificial Sequence: Synthetic peptide
QSISSY

SEQ ID NO: 36 - protein, 3 aa, Artificial Sequence
  Description of Artificial Sequence: Synthetic peptide
AAS

SEQ ID NO: 37 - protein, 9 aa, Artificial Sequence
  Description of Artificial Sequence: Synthetic peptide
QQSYSTPYT

SEQ ID NO: 38 - protein, 10 aa, Artificial Sequence
  Description of Artificial Sequence: Synthetic peptide
GDSVSSNSAT

SEQ ID NO: 39 - protein, 9 aa, Artificial Sequence
  Description of Artificial Sequence: Synthetic peptide
TYYRSKWYD

SEQ ID NO: 40 - protein, 11 aa, Artificial Sequence
  Description of Artificial Sequence: Synthetic peptide
AREGVAGDFDY

SEQ ID NO: 41 - DNA, 726 bp, Artificial Sequence
  Description of Artificial Sequence: Synthetic polynucleotide
caagttcagttgcagcagagtggccctgggcttgttaaaccatcacagacgctctcactgacctgtgccatctctggagacagtgtaagttctaactcagccgcgtggaattggattagacaatcaccaagccggggacttgaatggcttggtcggacgtactatagatctaagtggtataatgactacgcagtgtcagtgaaatcacggataaccataaaccctgacaccagcaaaaaccaattttctcttcagcttaattccgtcacgccagaagatacggccgtttactactgtgcgagggaaggtgatgacgcattggacatctggggtcaggggaccatggtgactgtctcttccggcggggggggtagtggagggggtggctcaggtggtggcgggtcagatatacaaatgacacagagccctagtagtctgagtgcttcagtgggcgaccgcgtaactataacctgtagagcatcccaaagcatttcccacttccttaattggtaccagcagaagccgggcacagcgcccaaactcctgatcaccactgcgagcggacttggttcaggtgttcctagccggtttagtgggtcaggtagcggtacagatttcactctcacgataaactcccttcagcctgaggacctggcgacatattactgtcaacaatcctataccaccccactgacattcggagggggcacaaaactggagatcaaa

SEQ ID NO: 42 - protein, 243 aa, Artificial Sequence
  Description of Artificial Sequence: Synthetic polypeptide
QVQLQQSGPGLVKPSQTLSLTCAISGDSVSSNSAAWNWIRQSPSRGLEWLGRTYYRSKWYNDYAVSVKSRITINPDTSKNQFSLQLNSVTPEDTAVYYCAREGDDALDIWGQGTMVTVSSGGGGSGGGGSGGGGSDIQMTQSPSSLSASVGDRVTITCRASQSISHFLNWYQQKPGTAPKLLITTASGLGSGVPSRFSGSGSGTDFTLTINSLQPEDLATYYCQQSYTTPLTFGGGTKLEIKR

SEQ ID NO: 43 - DNA, 1470 bp, Artificial Sequence
  Description of Artificial Sequence: Synthetic polynucleotide
atgcttctcctggtgacaagccttctgctctgtgagttaccacacccagcattcctcctgatcccacaagttcagttgcagcagagtggccctgggcttgttaaaccatcacagacgctctcactgacctgtgccatctctggagacagtgtaagttctaactcagccgcgtggaattggattagacaatcaccaagccggggacttgaatggcttggtcggacgtactatagatctaagtggtataatgactacgcagtgtcagtgaaatcacggataaccataaaccctgacaccagcaaaaaccaattttctcttcagcttaattccgtcacgccagaagatacggccgtttactactgtgcgagggaaggtgatgacgcattggacatctggggtcaggggaccatggtgactgtctcttccggcggggggggtagtggagggggtggctcaggtggtggcgggtcagatatacaaatgacacagagccctagtagtctgagtgcttcagtgggcgaccgcgtaactataacctgtagagcatcccaaagcatttcccacttccttaattggtaccagcagaagccgggcacagcgcccaaactcctgatcaccactgcgagcggacttggttcaggtgttcctagccggtttagtgggtcaggtagcggtacagatttcactctcacgataaactcccttcagcctgaggacctggcgacatattactgtcaacaatcctataccaccccactgacattcggagggggcacaaaactggagatcaaagcggccgcaactaccacccctgcccctcggccgccgactccggccccaaccatcgcaagccaacccctctccttgcgccccgaagcttgccgcccggccgcgggtggagccgtgcatacccgggggctggactttgcctgcgatatctacatttgggccccgctggccggcacttgcggcgtgctcctgctgtcgctggtcatcaccctttactgcaagaggggccggaagaagctgctttacatcttcaagcagccgttcatgcggcccgtgcagacgactcaggaagaggacggatgctcgtgcagattccctgaggaggaagaggggggatgcgaactgcgcgtcaagttctcacggtccgccgacgcccccgcatatcaacagggccagaatcagctctacaacgagctgaacctgggaaggagagaggagtacgacgtgctggacaagcgacgcggacgcgacccggagatgggggggaaaccacggcggaaaaaccctcaggaaggactgtacaacgaactccagaaagacaagatggcggaagcctactcagaaatcgggatgaagggagagcggaggaggggaaagggtcacgacgggctgtaccagggactgagcaccgccactaaggatacctacgatgccttgcatatgcaagcactcccaccccgg

SEQ ID NO: 44 - protein, 490 aa, Artificial Sequence
  Description of Artificial Sequence: Synthetic polypeptide
MLLLVTSLLLCELPHPAFLLIPQVQLQQSGPGLVKPSQTLSLTCAISGDSVSSNSAAWNWIRQSPSRGLEWLGRTYYRSKWYNDYAVSVKSRITINPDTSKNQFSLQLNSVTPEDTAVYYCAREGDDALDIWGQGTMVTVSSGGGGSGGGGSGGGGSDIQMTQSPSSLSASVGDRVTITCRASQSISHFLNWYQQKPGTAPKLLITTASGLGSGVPSRFSGSGSGTDFTLTINSLQPEDLATYYCQQSYTTPLTFGGGTKLEIKAAATTTPAPRPPTPAPTIASQPLSLRPEACRPAAGGAVHTRGLDFACDIYIWAPLAGTCGVLLLSLVITLYCKRGRKKLLYIFKQPFMRPVQTTQEEDGCSCRFPEEEEGGCELRVKFSRSADAPAYQQGQNQLYNELNLGRREEYDVLDKRRGRDPEMGGKPRRKNPQEGLYNELQKDKMAEAYSEIGMKGERRRGKGHDGLYQGLSTATKDTYDALHMQALPPR

SEQ ID NO: 45 - protein, 6 aa, Artificial Sequence
  Description of Artificial Sequence: Synthetic peptide
QSISHF

SEQ ID NO: 46 - protein, 3 aa, Artificial Sequence
  Description of Artificial Sequence: Synthetic peptide
TAS

SEQ ID NO: 47 - protein, 9 aa, Artificial Sequence
  Description of Artificial Sequence: Synthetic peptide
QQSYTTPLT

SEQ ID NO: 48 - protein, 10 aa, Artificial Sequence
  Description of Artificial Sequence: Synthetic peptide
GDSVSSNSAA

SEQ ID NO: 49 - protein, 9 aa, Artificial Sequence
  Description of Artificial Sequence: Synthetic peptide
TYYRSKWYN

SEQ ID NO: 50 - protein, 10 aa, Artificial Sequence
  Description of Artificial Sequence: Synthetic peptide
AREGDDALDI

SEQ ID NO: 51 - DNA, 732 bp, Artificial Sequence
  Description of Artificial Sequence: Synthetic polynucleotide
cagatacagttgcagcagtcaggtccaggactagtgaagccctcgcagaccctctcactcacctgtgccatctccggggacagtgtctctagcaacagtgctgcttggaactggatcaggcagtccccatcgagaggccttgagtggctgggaaggacatactacaggtccaagtggtataatgattatgcagtatctgtgaaaagtcgaataaccatcaacccagacacatccaagaaccagttctccctgcagctgaactctgtgactcccgaggacacggctgtgtattactgtgcccaagaggtacaacctgatgatgctttagatatctggggccaagggacaatggtcaccgtctcttcaggaggtggcgggtctggcggtggaggtagcggtggtggcggatccgacatccagatgacccagtctccatcttccgtgtctgcatctgtaggagacaaagtcaccatcacttgtcgggcgagtcaggatgttagcggctggttagcctggtatcagcagaaaccagggctagcccctcagctcctgatctctggtgcatccactttgcaaggtgaagtcccatcaaggttcagcggcagtggatctgggacagattttactctcaccatcagcagcctgcagcctgaagattttgccacttattattgtcaacaggctaaaaatttcccttacacttttggccaggggaccaagctggaaatcaaa

SEQ ID NO: 52 - protein, 244 aa, Artificial Sequence
  Description of Artificial Sequence: Synthetic polypeptide
QIQLQQSGPGLVKPSQTLSLTCAISGDSVSSNSAAWNWIRQSPSRGLEWLGRTYYRSKWYNDYAVSVKSRITINPDTSKNQFSLQLNSVTPEDTAVYYCAQEVQPDDALDIWGQGTMVTVSSGGGGSGGGGSGGGGSDIQMTQSPSSVSASVGDKVTITCRASQDVSGWLAWYQQKPGLAPQLLISGASTLQGEVPSRFSGSGSGTDFTLTISSLQPEDFATYYCQQAKNFPYTFGQGTKLEIK

SEQ ID NO: 53 - DNA, 1476 bp, Artificial Sequence
  Description of Artificial Sequence: Synthetic polynucleotide
atgttgttgcttgtcacaagccttcttctctgtgagcttccgcacccggctttcctgctgatcccgcagatacagcttcagcagtccggccccggtctggtaaagccgtcccaaacgctttcactcacatgcgcgatctctggtgattctgtgtcatccaacagcgcagcatggaattggatccgccaatcacccagtagaggcttggagtggttgggccggacttattatcgaagtaagtggtacaatgattatgcagtctcagttaaatccaggatcactattaacccagatacaagtaaaaaccagttctcattgcaacttaattccgtaactccggaggacactgcagtatattactgcgctcaggaggtgcagcctgatgatgctctggacatttggggacaaggcacgatggtcacggttagttccggggggggaggttctggcggaggtggtagtggggggggcggcagtgacatccagatgacacagagtcccagcagcgtgtctgcgtcagtcggggataaggtaacaattacgtgtagagcgagccaggacgtttccgggtggctggcgtggtaccaacaaaaacccggtctcgctccgcagttgctcatctctggagcgtccacccttcagggagaggtgcctagcagattttctgggtctggatccggcacggattttacacttacgatttcctctcttcaacccgaagattttgctacttactattgccagcaggccaaaaacttcccgtacacgtttggacagggcacaaagttggaaattaaggcggccgcaactaccacccctgcccctcggccgccgactccggccccaaccatcgcaagccaacccctctccttgcgccccgaagcttgccgcccggccgcgggtggagccgtgcatacccgggggctggactttgcctgcgatatctacatttgggccccgctggccggcacttgcggcgtgctcctgctgtcgctggtcatcaccctttactgcaagaggggccggaagaagctgctttacatcttcaagcagccgttcatgcggcccgtgcagacgactcaggaagaggacggatgctcgtgcagattccctgaggaggaagaggggggatgcgaactgcgcgtcaagttctcacggtccgccgacgcccccgcatatcaacagggccagaatcagctctacaacgagctgaacctgggaaggagagaggagtacgacgtgctggacaagcgacgcggacgcgacccggagatgggggggaaaccacggcggaaaaaccctcaggaaggactgtacaacgaactccagaaagacaagatggcggaagcctactcagaaatcgggatgaagggagagcggaggaggggaaagggtcacgacgggctgtaccagggactgagcaccgccactaaggatacctacgatgccttgcatatgcaagcactcccaccccgg

SEQ ID NO: 54 - protein, 492 aa, Artificial Sequence
  Description of Artificial Sequence: Synthetic polypeptide
MLLLVTSLLLCELPHPAFLLIPQIQLQQSGPGLVKPSQTLSLTCAISGDSVSSNSAAWNWIRQSPSRGLEWLGRTYYRSKWYNDYAVSVKSRITINPDTSKNQFSLQLNSVTPEDTAVYYCAQEVQPDDALDIWGQGTMVTVSSGGGGSGGGGSGGGGSDIQMTQSPSSVSASVGDKVTITCRASQDVSGWLAWYQQKPGLAPQLLISGASTLQGEVPSRFSGSGSGTDFTLTISSLQPEDFATYYCQQAKNFPYTFGQGTKLEIKAAATTTPAPRPPTPAPTIASQPLSLRPEACRPAAGGAVHTRGLDFACDIYIWAPLAGTCGVLLLSLVITLYCKRGRKKLLYIFKQPFMRPVQTTQEEDGCSCRFPEEEEGGCELRVKFSRSADAPAYQQGQNQLYNELNLGRREEYDVLDKRRGRDPEMGGKPRRKNPQEGLYNELQKDKMAEAYSEIGMKGERRRGKGHDGLYQGLSTATKDTYDALHMQALPPR

SEQ ID NO: 55 - protein, 6 aa, Artificial Sequence
  Description of Artificial Sequence: Synthetic peptide
QDVSGW

SEQ ID NO: 56 - protein, 3 aa, Artificial Sequence
  Description of Artificial Sequence: Synthetic peptide
GAS

SEQ ID NO: 57 - protein, 9 aa, Artificial Sequence
  Description of Artificial Sequence: Synthetic peptide
QQAKNFPYT

SEQ ID NO: 58 - protein, 10 aa, Artificial Sequence
  Description of Artificial Sequence: Synthetic peptide
GDSVSSNSAA

SEQ ID NO: 59 - protein, 9 aa, Artificial Sequence
  Description of Artificial Sequence: Synthetic peptide
TYYRSKWYN

SEQ ID NO: 60 - protein, 12 aa, Artificial Sequence
  Description of Artificial Sequence: Synthetic peptide
AQEVQPDDALDI

SEQ ID NO: 61 - DNA, 732 bp, Artificial Sequence
  Description of Artificial Sequence: Synthetic polynucleotide
caagtacagttgcagcagtcaggacctggccttgtgaaaccatcccaaactctcagcctcacgtgtgctatttctggtgactcagtaagtagcaatagcgctgcttggaactggatcagacaatctccctccaggggtctcgaatggctggggcgaacctattaccgatctaaatggtataacgattatgcagtatccgtgaaatccaggattacaatcaacccagatacgttcaagaatcaattctctcttcagctcaactccgtaactccagaggacactgcggtatattattgcgcccaagaagtcgagccacacgatgccctcgatatctggggtcaaggtaccatggttacagttagtagtgggggtgggggaagcgggggcggtgggtccggtggcgggggttcagacatcaagatgacccaatccccaagctctgtttcagcatccgtgggcgataaggtaaccattacatgcagagcgagtcaggacgtttcagggtggctggcttggtaccagcaaaaaccgggactcgcaccgcagctgttgattttcggcgccagtacgcttcagggcgaagtaccgtccaggttcagtgggtcaggttctggcaccgattttacgctcacgatatccagtctccaaccggaggattttgctacttattactgccagcaggctaagtattttccatacacatttggccaggggacaaagttggagatcaaa

SEQ ID NO: 62 - protein, 244 aa, Artificial Sequence
  Description of Artificial Sequence: Synthetic polypeptide
QVQLQQSGPGLVKPSQTLSLTCAISGDSVSSNSAAWNWIRQSPSRGLEWLGRTYYRSKWYNDYAVSVKSRITINPDTFKNQFSLQLNSVTPEDTAVYYCAQEVEPHDALDIWGQGTMVTVSSGGGGSGGGGSGGGGSDIKMTQSPSSVSASVGDKVTITCRASQDVSGWLAWYQQKPGLAPQLLIFGASTLQGEVPSRFSGSGSGTDFTLTISSLQPEDFATYYCQQAKYFPYTFGQGTKLEIK

SEQ ID NO: 63 - DNA, 1476 bp, Artificial Sequence
  Description of Artificial Sequence: Synthetic polynucleotide
atgctgcttttggtaacttccctccttttgtgcgagctgccccatccagcgttcctcctcatccctcaagtacagttgcagcagtcaggacctggccttgtgaaaccatcccaaactctcagcctcacgtgtgctatttctggtgactcagtaagtagcaatagcgctgcttggaactggatcagacaatctccctccaggggtctcgaatggctggggcgaacctattaccgatctaaatggtataacgattatgcagtatccgtgaaatccaggattacaatcaacccagatacgttcaagaatcaattctctcttcagctcaactccgtaactccagaggacactgcggtatattattgcgcccaagaagtcgagccacacgatgccctcgatatctggggtcaaggtaccatggttacagttagtagtgggggtgggggaagcgggggcggtgggtccggtggcgggggttcagacatcaagatgacccaatccccaagctctgtttcagcatccgtgggcgataaggtaaccattacatgcagagcgagtcaggacgtttcagggtggctggcttggtaccagcaaaaaccgggactcgcaccgcagctgttgattttcggcgccagtacgcttcagggcgaagtaccgtccaggttcagtgggtcaggttctggcaccgattttacgctcacgatatccagtctccaaccggaggattttgctacttattactgccagcaggctaagtattttccatacacatttggccaggggacaaagttggagatcaaagcggccgcaactaccacccctgcccctcggccgccgactccggccccaaccatcgcaagccaacccctctccttgcgccccgaagcttgccgcccggccgcgggtggagccgtgcatacccgggggctggactttgcctgcgatatctacatttgggccccgctggccggcacttgcggcgtgctcctgctgtcgctggtcatcaccctttactgcaagaggggccggaagaagctgctttacatcttcaagcagccgttcatgcggcccgtgcagacgactcaggaagaggacggatgctcgtgcagattccctgaggaggaagaggggggatgcgaactgcgcgtcaagttctcacggtccgccgacgcccccgcatatcaacagggccagaatcagctctacaacgagctgaacctgggaaggagagaggagtacgacgtgctggacaagcgacgcggacgcgacccggagatgggggggaaaccacggcggaaaaaccctcaggaaggactgtacaacgaactccagaaagacaagatggcggaagcctactcagaaatcgggatgaagggagagcggaggaggggaaagggtcacgacgggctgtaccagggactgagcaccgccactaaggatacctacgatgccttgcatatgcaagcactcccaccccgg

SEQ ID NO: 64 - protein, 492 aa, Artificial Sequence
  Description of Artificial Sequence: Synthetic polypeptide
MLLLVTSLLLCELPHPAFLLIPQVQLQQSGPGLVKPSQTLSLTCAISGDSVSSNSAAWNWIRQSPSRGLEWLGRTYYRSKWYNDYAVSVKSRITINPDTFKNQFSLQLNSVTPEDTAVYYCAQEVEPHDALDIWGQGTMVTVSSGGGGSGGGGSGGGGSDIKMTQSPSSVSASVGDKVTITCRASQDVSGWLAWYQQKPGLAPQLLIFGASTLQGEVPSRFSGSGSGTDFTLTISSLQPEDFATYYCQQAKYFPYTFGQGTKLEIKAAATTTPAPRPPTPAPTIASQPLSLRPEACRPAAGGAVHTRGLDFACDIYIWAPLAGTCGVLLLSLVITLYCKRGRKKLLYIFKQPFMRPVQTTQEEDGCSCRFPEEEEGGCELRVKFSRSADAPAYQQGQNQLYNELNLGRREEYDVLDKRRGRDPEMGGKPRRKNPQEGLYNELQKDKMAEAYSEIGMKGERRRGKGHDGLYQGLSTATKDTYDALHMQALPPR

SEQ ID NO: 65 - protein, 6 aa, Artificial Sequence
  Description of Artificial Sequence: Synthetic peptide
QDVSGW

SEQ ID NO: 66 - protein, 3 aa, Artificial Sequence
  Description of Artificial Sequence: Synthetic peptide
GAS

SEQ ID NO: 67 - protein, 9 aa, Artificial Sequence
  Description of Artificial Sequence: Synthetic peptide
QQAKYFPYT

SEQ ID NO: 68 - protein, 10 aa, Artificial Sequence
  Description of Artificial Sequence: Synthetic peptide
GDSVSSNSAA

SEQ ID NO: 69 - protein, 9 aa, Artificial Sequence
  Description of Artificial Sequence: Synthetic peptide
TYYRSKWYN

SEQ ID NO: 70 - protein, 12 aa, Artificial Sequence
  Description of Artificial Sequence: Synthetic peptide
AQEVEPHDALDI

SEQ ID NO: 71 - DNA, 732 bp, Artificial Sequence
  Description of Artificial Sequence: Synthetic polynucleotide
caggtacagctgcagcagtcaggtccaggactggtgaagccctcgcagaccctctcactcacctgtgccatctccggggacagtgtctctagcaacagtgctgcttggaactggatcaggcagtccccatcgagaggccttgagtggctgggaaggacatactacaggtccaagtggtataatgattatgcagtatctgtgaaaagtcgaataaccatcaacccagacacatccaagaaccagttctccctgcagctgaactctgtgactcccgaggacacggctgtgtattactgtgcccaagaggtagaacctcatgatgctcttgatatctggggccaagggacaatggtcaccgtctcttcaggaggtggcgggtctggcggaggcggtagcggtggtggcggatccgacatccagatgacgcagtctccatcatccgtgtctgcatctgtaggagacaaagtcaccatcacttgtcgggcgagtcaggatgttagcggctggttagcctggtatcaacagaaaccagggctagcccctcagctcctgatctttggtgcatccactttgcaaggtgaagtcccatcaaggttcagcggcagtggatctgggacagattttactctcaccatcagcagcctgcagcctgaagattttgccacttattattgtcaacaggctaaatatttcccttacacttttggccaggggaccaagctggagatcaaa

SEQ ID NO: 72 - protein, 244 aa, Artificial Sequence
  Description of Artificial Sequence: Synthetic polypeptide
QVQLQQSGPGLVKPSQTLSLTCAISGDSVSSNSAAWNWIRQSPSRGLEWLGRTYYRSKWYNDYAVSVKSRITINPDTSKNQFSLQLNSVTPEDTAVYYCAQEVEPHDALDIWGQGTMVTVSSGGGGSGGGGSGGGGSDIQMTQSPSSVSASVGDKVTITCRASQDVSGWLAWYQQKPGLAPQLLIFGASTLQGEVPSRFSGSGSGTDFTLTISSLQPEDFATYYCQQAKYFPYTFGQGTKLEIK

SEQ ID NO: 73 - DNA, 1476 bp, Artificial Sequence
  Description of Artificial Sequence: Synthetic polynucleotide
atgctgctcctcgtaacctctcttcttctttgtgagttgccacatccagcatttcttctgatacctcaagttcaactccagcagagtggtccaggtttggtaaaacccagccagactctctcattgacgtgtgccatatcaggtgattcagtttcctctaatagcgcggcatggaattggatcaggcaaagccctagtcgcgggctggagtggctcggccggacatactaccgctcaaagtggtacaacgactacgccgtcagcgtaaaatctcggattaccattaacccggatacttccaaaaaccaattctccctgcagcttaacagtgtcacgccggaagatacggccgtttattactgcgcacaagaggtggaaccgcacgacgccctcgatatctggggccaaggcactatggtgaccgtcagtagcggaggggggggttccggaggaggcggctctggtggcggaggatctgatatccaaatgacccaatcaccgtcttcagtatcagcttctgttggtgacaaagttacgattacctgtcgagcgtcacaggacgtttctggttggttggcttggtatcagcaaaaaccagggcttgcgcctcagttgcttatttttggggcatctactttgcagggagaggtgccctcccggttctccggcagtgggagcggcaccgattttacacttaccatctcttccttgcaacccgaagactttgcgacgtactattgccagcaggcaaagtattttccctacacttttggacaagggactaaacttgaaatcaaggcggccgcaactaccacccctgcccctcggccgccgactccggccccaaccatcgcaagccaacccctctccttgcgccccgaagcttgccgcccggccgcgggtggagccgtgcatacccgggggctggactttgcctgcgatatctacatttgggccccgctggccggcacttgcggcgtgctcctgctgtcgctggtcatcaccctttactgcaagaggggccggaagaagctgctttacatcttcaagcagccgttcatgcggcccgtgcagacgactcaggaagaggacggatgctcgtgcagattccctgaggaggaagaggggggatgcgaactgcgcgtcaagttctcacggtccgccgacgcccccgcatatcaacagggccagaatcagctctacaacgagctgaacctgggaaggagagaggagtacgacgtgctggacaagcgacgcggacgcgacccggagatgggggggaaaccacggcggaaaaaccctcaggaaggactgtacaacgaactccagaaagacaagatggcggaagcctactcagaaatcgggatgaagggagagcggaggaggggaaagggtcacgacgggctgtaccagggactgagcaccgccactaaggatacctacgatgccttgcatatgcaagcactcccaccccgg

SEQ ID NO: 74 - protein, 492 aa, Artificial Sequence
  Description of Artificial Sequence: Synthetic polypeptide
MLLLVTSLLLCELPHPAFLLIPQVQLQQSGPGLVKPSQTLSLTCAISGDSVSSNSAAWNWIRQSPSRGLEWLGRTYYRSKWYNDYAVSVKSRITINPDTSKNQFSLQLNSVTPEDTAVYYCAQEVEPHDALDIWGQGTMVTVSSGGGGSGGGGSGGGGSDIQMTQSPSSVSASVGDKVTITCRASQDVSGWLAWYQQKPGLAPQLLIFGASTLQGEVPSRFSGSGSGTDFTLTISSLQPEDFATYYCQQAKYFPYTFGQGTKLEIKAAATTTPAPRPPTPAPTIASQPLSLRPEACRPAAGGAVHTRGLDFACDIYIWAPLAGTCGVLLLSLVITLYCKRGRKKLLYIFKQPFMRPVQTTQEEDGCSCRFPEEEEGGCELRVKFSRSADAPAYQQGQNQLYNELNLGRREEYDVLDKRRGRDPEMGGKPRRKNPQEGLYNELQKDKMAEAYSEIGMKGERRRGKGHDGLYQGLSTATKDTYDALHMQALPPR

SEQ ID NO: 75 - protein, 6 aa, Artificial Sequence
  Description of Artificial Sequence: Synthetic peptide
QDVSGW

SEQ ID NO: 76 - protein, 3 aa, Artificial Sequence
  Description of Artificial Sequence: Synthetic peptide
GAS

SEQ ID NO: 77 - protein, 9 aa, Artificial Sequence
  Description of Artificial Sequence: Synthetic peptide
QQAKYFPYT

SEQ ID NO: 78 - protein, 10 aa, Artificial Sequence
  Description of Artificial Sequence: Synthetic peptide
GDSVSSNSAA

SEQ ID NO: 79 - protein, 9 aa, Artificial Sequence
  Description of Artificial Sequence: Synthetic peptide
TYYRSKWYN

SEQ ID NO: 80 - protein, 12 aa, Artificial Sequence
  Description of Artificial Sequence: Synthetic peptide
AQEVEPHDALDI

SEQ ID NO: 81 - DNA, 732 bp, Artificial Sequence
  Description of Artificial Sequence: Synthetic polynucleotide
caggtacagctgcagcagtcaggtccaggactggtgaagccctcgcagaccctctcactcacctgtgccatctccggggacagtgtctctagcaacagtgctgcttggaactggatcaggcagtccccatcgagaggccttgagtggctgggaaggacatactacaggtccaagtggtataatgattatgcagtatctgtgaaaagtcgaataaccatcaacccagacacattcaagaaccagttctccctgcagctgaactctgtgactcccgaggacacggctgtgtattactgtgcccaagaggtagaacctcatgatgctcttgatatctggggccaagggacaatggtcaccgtctcttcaggaggtggcgggtctggcggtggaggtagcggtggtggcggatccgacatcaagatgacccagtctccatcttccgtgtctgcatctgtaggagacaaagtcaccatcacttgtcgggcgagtcaggatgttagcggctggttagcctggtatcagcagaaaccagggctagcccctcagctcctgatctttggtgcatccactttgcaaggtgaagtcccatcaaggttcagcggcagtggatctgggacagattttactctcaccatcagcagcctgcagcctgaagattttgccacttattattgtcaacaggctaaatatttcccttacacttttggccaggggaccaagctggaaatcaaa

SEQ ID NO: 82 - protein, 244 aa, Artificial Sequence; identical to SEQ ID NO: 62
  Description of Artificial Sequence: Synthetic polypeptide

SEQ ID NO: 83 - DNA, 1476 bp, Artificial Sequence
  Description of Artificial Sequence: Synthetic polynucleotide
atgcttcttttggtgacttcccttttgctgtgcgagttgccacaccccgccttcctgcttattccccaagtccagctccaacaatccggacccggacttgttaagccgtctcagacgttgtcactcacatgcgccatcagtggcgatagcgtgtccagcaacagtgccgcatggaattggatacgacagagcccttcccgaggattggaatggctgggacgaacgtactataggtccaagtggtataacgactacgcggtgtcagttaaatctcggattactataaatcccgacacttttaagaatcagttttccctgcaactcaattcagtcacaccggaagatacggcagtgtactattgcgctcaagaagttgagccacatgatgcgctggatatttggggtcaggggactatggtgacggtaagcagtgggggcgggggcagtggcggaggtggcagcgggggcggtggaagcgacattaagatgactcagtctccgtcttcagtttccgcctccgtaggggacaaggttacaattacttgtcgcgcatctcaggatgtctcaggttggctggcttggtatcaacagaagcctggcctcgcccctcagcttctcatattcggggctagtaccctgcaaggagaagtcccgagcaggttttccggttcagggtccgggacagactttaccttgaccatcagctccctgcaaccggaggacttcgcgacctactattgtcaacaggcgaagtacttcccctacacgttcgggcaagggactaagctcgaaatcaaggcggccgcaactaccacccctgcccctcggccgccgactccggccccaaccatcgcaagccaacccctctccttgcgccccgaagcttgccgcccggccgcgggtggagccgtgcatacccgggggctggactttgcctgcgatatctacatttgggccccgctggccggcacttgcggcgtgctcctgctgtcgctggtcatcaccctttactgcaagaggggccggaagaagctgctttacatcttcaagcagccgttcatgcggcccgtgcagacgactcaggaagaggacggatgctcgtgcagattccctgaggaggaagaggggggatgcgaactgcgcgtcaagttctcacggtccgccgacgcccccgcatatcaacagggccagaatcagctctacaacgagctgaacctgggaaggagagaggagtacgacgtgctggacaagcgacgcggacgcgacccggagatgggggggaaaccacggcggaaaaaccctcaggaaggactgtacaacgaactccagaaagacaagatggcggaagcctactcagaaatcgggatgaagggagagcggaggaggggaaagggtcacgacgggctgtaccagggactgagcaccgccactaaggatacctacgatgccttgcatatgcaagcactcccaccccgg

SEQ ID NO: 84 - protein, 492 aa, Artificial Sequence; identical to SEQ ID NO: 64
  Description of Artificial Sequence: Synthetic polypeptide

SEQ ID NO: 85 - protein, 6 aa, Artificial Sequence
  Description of Artificial Sequence: Synthetic peptide
QDVSGW

SEQ ID NO: 86 - protein, 3 aa, Artificial Sequence
  Description of Artificial Sequence: Synthetic peptide
GAS

SEQ ID NO: 87 - protein, 9 aa, Artificial Sequence
  Description of Artificial Sequence: Synthetic peptide
QQAKYFPYT

SEQ ID NO: 88 - protein, 10 aa, Artificial Sequence
  Description of Artificial Sequence: Synthetic peptide
GDSVSSNSAA

SEQ ID NO: 89 - protein, 9 aa, Artificial Sequence
  Description of Artificial Sequence: Synthetic peptide
TYYRSKWYN

SEQ ID NO: 90 - protein, 12 aa, Artificial Sequence
  Description of Artificial Sequence: Synthetic peptide
AQEVEPHDALDI

SEQ ID NO: 91 - DNA, 732 bp, Artificial Sequence
  Description of Artificial Sequence: Synthetic polynucleotide
caggtacagctgcagcagtcaggtccaggactggtgaagccctcgcagaccctctcactcacctgtgccatctccggggacagtgtctctagcaacagtgctgcttggaactggatcaggcagtccccatcgagaggccttgagtggctgggaaggacatactacaggtccaagtggtataatgattatgcagtatctgtgaaaagtcgaataaccatcaacccagacacatccaagaaccagttctccctgcagctgaactctgtgactcccgaggatacggctgtgtattactgtgcccaagaggtacaacctgatgatgcttttgatatctggggccaagggacaatgatcaccgtctcttcaggaggtggcgggtctggcggtggaggtagcggtggtggcggatccgacatccagatgacccagtctccatcttccgtgtctgcatctgtaggagacaaagtcaccatcacttgtcgggcgagtcaggatgttagcggctggttagcctggtatcagcagaaaccagggctagcccctcagctcctgatctctggtgcatccactttgcaaggtggagtcccatcaaggttcagcggcagtggatctgggacagattttactctcaccatcagcagcctgcagcctgaagattttgccacttattattgtcaacaggctaaaaatttcccttacacttttggtcaggggaccaagctggaaatcaaa

SEQ ID NO: 92 - protein, 244 aa, Artificial Sequence
  Description of Artificial Sequence: Synthetic polypeptide
QVQLQQSGPGLVKPSQTLSLTCAISGDSVSSNSAAWNWIRQSPSRGLEWLGRTYYRSKWYNDYAVSVKSRITINPDTSKNQFSLQLNSVTPEDTAVYYCAQEVQPDDAFDIWGQGTMITVSSGGGGSGGGGSGGGGSDIQMTQSPSSVSASVGDKVTITCRASQDVSGWLAWYQQKPGLAPQLLISGASTLQGGVPSRFSGSGSGTDFTLTISSLQPEDFATYYCQQAKNFPYTFGQGTKLEIK

SEQ ID NO: 93 - DNA, 1476 bp, Artificial Sequence
  Description of Artificial Sequence: Synthetic polynucleotide
atgcttcttttggtgacttcccttttgctgtgcgagttgccacaccccgccttcctgcttattccccaagtacaactccagcaatcagggcctggccttgtcaagccgagtcaaaccttgagtttgacgtgtgccatcagcggtgactctgtcagttcaaactccgcagcttggaactggattcggcagtccccctccaggggcctcgaatggcttggacggacgtactacagatcaaaatggtacaacgactacgcagtcagtgtaaaatcaaggattacgataaaccctgatacgagtaaaaaccagttctctctccaactgaacagcgtcacaccggaagatacagccgtgtattactgtgctcaggaagtgcaacctgacgacgcatttgacatctggggtcagggcacgatgatcaccgtgagtagtggaggaggaggcagtgggggaggcggttctggcgggggtgggtctgatatacagatgacacagagtccctcctcagtttccgcctctgttggagataaggtgacaattacatgcagggcgtcccaagatgtttctggatggctcgcatggtaccaacagaagccaggactcgcccctcagctcctcattagcggcgctagcactctccaagggggagtaccgagcaggttctctgggtccggaagtgggacggactttaccctgacaatatcctcccttcagccagaagacttcgcaacctactattgccaacaggcgaaaaatttcccttacacgttcggccaaggaactaaacttgaaatcaaggcggccgcaactaccacccctgcccctcggccgccgactccggccccaaccatcgcaagccaacccctctccttgcgccccgaagcttgccgcccggccgcgggtggagccgtgcatacccgggggctggactttgcctgcgatatctacatttgggccccgctggccggcacttgcggcgtgctcctgctgtcgctggtcatcaccctttactgcaagaggggccggaagaagctgctttacatcttcaagcagccgttcatgcggcccgtgcagacgactcaggaagaggacggatgctcgtgcagattccctgaggaggaagaggggggatgcgaactgcgcgtcaagttctcacggtccgccgacgcccccgcatatcaacagggccagaatcagctctacaacgagctgaacctgggaaggagagaggagtacgacgtgctggacaagcgacgcggacgcgacccggagatgggggggaaaccacggcggaaaaaccctcaggaaggactgtacaacgaactccagaaagacaagatggcggaagcctactcagaaatcgggatgaagggagagcggaggaggggaaagggtcacgacgggctgtaccagggactgagcaccgccactaaggatacctacgatgccttgcatatgcaagcactcccaccccgg

SEQ ID NO: 94 - protein, 492 aa, Artificial Sequence
  Description of Artificial Sequence: Synthetic polypeptide
MLLLVTSLLLCELPHPAFLLIPQVQLQQSGPGLVKPSQTLSLTCAISGDSVSSNSAAWNWIRQSPSRGLEWLGRTYYRSKWYNDYAVSVKSRITINPDTSKNQFSLQLNSVTPEDTAVYYCAQEVQPDDAFDIWGQGTMITVSSGGGGSGGGGSGGGGSDIQMTQSPSSVSASVGDKVTITCRASQDVSGWLAWYQQKPGLAPQLLISGASTLQGGVPSRFSGSGSGTDFTLTISSLQPEDFATYYCQQAKNFPYTFGQGTKLEIKAAATTTPAPRPPTPAPTIASQPLSLRPEACRPAAGGAVHTRGLDFACDIYIWAPLAGTCGVLLLSLVITLYCKRGRKKLLYIFKQPFMRPVQTTQEEDGCSCRFPEEEEGGCELRVKFSRSADAPAYQQGQNQLYNELNLGRREEYDVLDKRRGRDPEMGGKPRRKNPQEGLYNELQKDKMAEAYSEIGMKGERRRGKGHDGLYQGLSTATKDTYDALHMQALPPR

SEQ ID NO: 95 - protein, 6 aa, Artificial Sequence
  Description of Artificial Sequence: Synthetic peptide
QDVSGW

SEQ ID NO: 96 - protein, 3 aa, Artificial Sequence
  Description of Artificial Sequence: Synthetic peptide
GAS

SEQ ID NO: 97 - protein, 9 aa, Artificial Sequence
  Description of Artificial Sequence: Synthetic peptide
QQAKNFPYT

SEQ ID NO: 98 - protein, 10 aa, Artificial Sequence
  Description of Artificial Sequence: Synthetic peptide
GDSVSSNSAA

SEQ ID NO: 99 - protein, 9 aa, Artificial Sequence
  Description of Artificial Sequence: Synthetic peptide
TYYRSKWYN

SEQ ID NO: 100 - protein, 12 aa, Artificial Sequence
  Description of Artificial Sequence: Synthetic peptide
AQEVQPDDAFDI

SEQ ID NO: 101 - DNA, 732 bp, Artificial Sequence
  Description of Artificial Sequence: Synthetic polynucleotide
caggtacagctgcagcagtcaggtccaggactggtgaagccctcgcagaccctctcactcacctgtgccatctccggggacagtgtctctagcaacagtgctgcttggaactggatcaggcagtccccatcgagaggccttgagtggctgggaaggacatactacaggtccaagtggtataatgattatgcagtatctgtgaaaagtcgaataaccatcaacccagacacatccaagaaccagttctccctgcagctgaactctgtgactcccgaggacacggctgtgtattactgtgcccaagaggtagaacctcaggatgcttttgatatctggggccaagggacaatggtcaccgtctcttcaggaggtggcgggtctggtggtggcggtagcggtggtggcggatccgacatccagatgacccagtctccatcttccgtgtctgcatctgtaggagacaaagtcaccatcacttgtcgggcgagtcaggatgttagcggctggttagcctggtatcagcagaaaccagggctagcccctcagctcctgatctttggtgcatccactctgcaaggtgaagtcccatcaaggttcagtggcagtggatctgggacagattttactctcaccatcagcagcctgcagcctgaagattttgccacttattattgtcaacaggctaaatatttcccttacacttttggcccggggaccaagctggaaatcaaa

SEQ ID NO: 102 - protein, 244 aa, Artificial Sequence
  Description of Artificial Sequence: Synthetic polypeptide
QVQLQQSGPGLVKPSQTLSLTCAISGDSVSSNSAAWNWIRQSPSRGLEWLGRTYYRSKWYNDYAVSVKSRITINPDTSKNQFSLQLNSVTPEDTAVYYCAQEVEPQDAFDIWGQGTMVTVSSGGGGSGGGGSGGGGSDIQMTQSPSSVSASVGDKVTITCRASQDVSGWLAWYQQKPGLAPQLLIFGASTLQGEVPSRFSGSGSGTDFTLTISSLQPEDFATYYCQQAKYFPYTFGPGTKLEIK

SEQ ID NO: 103 - DNA, 1476 bp, Artificial Sequence
  Description of Artificial Sequence: Synthetic polynucleotide
atgcttcttttggtgacttcccttttgctgtgcgagttgccacaccccgccttcctgcttattccccaagtgcagttgcaacagtctggaccaggcctcgtaaaaccttctcaaactttgtcactcacttgtgccatctcaggggacagtgtcagttccaacagtgcggcatggaattggattaggcaatccccctctcgaggtctggaatggcttgggcggacttactaccgaagtaagtggtacaacgattatgcagtttctgtaaaatcacgaatcactataaatccggacacttctaagaatcagttctctttgcagcttaactctgttactcctgaagacacagccgtatattactgtgctcaagaggtagagccgcaagatgccttcgacatctggggccaagggactatggtgacagtaagctccggaggtgggggatcagggggaggtgggtccggtggtggtggctctgacatacagatgacacagtcccctagctctgtgtcagcaagtgtcggtgacaaggttacgataacgtgcagggccagtcaagatgtgtcaggatggttggcgtggtaccaacagaaacccggcttggcaccgcagcttttgatattcggcgcgtccacactccaaggcgaagtgccttctcggttttctggaagcggcagcgggacggactttactttgacaatatcctccctccaacccgaggatttcgcgacgtattattgccagcaagcaaaatacttcccatacaccttcgggcctgggaccaaactggagatcaaagcggccgcaactaccacccctgcccctcggccgccgactccggccccaaccatcgcaagccaacccctctccttgcgccccgaagcttgccgcccggccgcgggtggagccgtgcatacccgggggctggactttgcctgcgatatctacatttgggccccgctggccggcacttgcggcgtgctcctgctgtcgctggtcatcaccctttactgcaagaggggccggaagaagctgctttacatcttcaagcagccgttcatgcggcccgtgcagacgactcaggaagaggacggatgctcgtgcagattccctgaggaggaagaggggggatgcgaactgcgcgtcaagttctcacggtccgccgacgcccccgcatatcaacagggccagaatcagctctacaacgagctgaacctgggaaggagagaggagtacgacgtgctggacaagcgacgcggacgcgacccggagatgggggggaaaccacggcggaaaaaccctcaggaaggactgtacaacgaactccagaaagacaagatggcggaagcctactcagaaatcgggatgaagggagagcggaggaggggaaagggtcacgacgggctgtaccagggactgagcaccgccactaaggatacctacgatgccttgcatatgcaagcactcccaccccgg

SEQ ID NO: 104 - protein, 492 aa, Artificial Sequence
  Description of Artificial Sequence: Synthetic polypeptide
MLLLVTSLLLCELPHPAFLLIPQVQLQQSGPGLVKPSQTLSLTCAISGDSVSSNSAAWNWIRQSPSRGLEWLGRTYYRSKWYNDYAVSVKSRITINPDTSKNQFSLQLNSVTPEDTAVYYCAQEVEPQDAFDIWGQGTMVTVSSGGGGSGGGGSGGGGSDIQMTQSPSSVSASVGDKVTITCRASQDVSGWLAWYQQKPGLAPQLLIFGASTLQGEVPSRFSGSGSGTDFTLTISSLQPEDFATYYCQQAKYFPYTFGPGTKLEIKAAATTTPAPRPPTPAPTIASQPLSLRPEACRPAAGGAVHTRGLDFACDIYIWAPLAGTCGVLLLSLVITLYCKRGRKKLLYIFKQPFMRPVQTTQEEDGCSCRFPEEEEGGCELRVKFSRSADAPAYQQGQNQLYNELNLGRREEYDVLDKRRGRDPEMGGKPRRKNPQEGLYNELQKDKMAEAYSEIGMKGERRRGKGHDGLYQGLSTATKDTYDALHMQALPPR

SEQ ID NO: 105 - protein, 6 aa, Artificial Sequence
  Description of Artificial Sequence: Synthetic peptide
QDVSGW

SEQ ID NO: 106 - protein, 3 aa, Artificial Sequence
  Description of Artificial Sequence: Synthetic peptide
GAS

SEQ ID NO: 107 - protein, 9 aa, Artificial Sequence
  Description of Artificial Sequence: Synthetic peptide
QQAKYFPYT

SEQ ID NO: 108 - protein, 10 aa, Artificial Sequence
  Description of Artificial Sequence: Synthetic peptide
GDSVSSNSAA

SEQ ID NO: 109 - protein, 9 aa, Artificial Sequence
  Description of Artificial Sequence: Synthetic peptide
TYYRSKWYN

SEQ ID NO: 110 - protein, 12 aa, Artificial Sequence
  Description of Artificial Sequence: Synthetic peptide
AQEVEPQDAFDI

SEQ ID NO: 111 - DNA, 732 bp, Artificial Sequence
  Description of Artificial Sequence: Synthetic polynucleotide
caggtacagctgcagcagtcaggtccaggactggtgaagcactcgcagaccctctcactcacctgtgccatctccggggacagtgtctctagcaacagtgctgcttggaactggatcaggcagtccccatcgagaggccttgagtggctgggaaggacatactacaggtccaagtggtataatgattatgcagtatctgtgaaaagtcgaataaccatcaacccagacacatccaagaaccagttctccctgcagttgaactctgtgactcccgaggacacggctgtgtattactgtgcccaagaggtagaacctcatgatgcttttgatatctggggccaagggacaatggtcaccgtctcttcaggaggtggcgggtctggcggtggaggtagcggtggtggcggatccgacatccagatgacccagtctccatcttccgtgtatgcatctgtaggagacaaagtcaccatcacttgtcgggcgagtcaggatgttagcggctggttagcctggtatcagcagaaaccagggctagcccctcagctcctgatctctggtgcatccactttgcaaggtgaagtcccatcaaggttcagcggcagtggatctgggacagattttactctcaccatcagcagcctgcagcctgaagattttgccacttattattgtcaacaggctaaatatttcccttacacttttggccaggggaccaagctggaaatcaaa

SEQ ID NO: 112 - protein, 244 aa, Artificial Sequence
  Description of Artificial Sequence: Synthetic polypeptide
QVQLQQSGPGLVKHSQTLSLTCAISGDSVSSNSAAWNWIRQSPSRGLEWLGRTYYRSKWYNDYAVSVKSRITINPDTSKNQFSLQLNSVTPEDTAVYYCAQEVEPHDAFDIWGQGTMVTVSSGGGGSGGGGSGGGGSDIQMTQSPSSVYASVGDKVTITCRASQDVSGWLAWYQQKPGLAPQLLISGASTLQGEVPSRFSGSGSGTDFTLTISSLQPEDFATYYCQQAKYFPYTFGQGTKLEIK

SEQ ID NO: 113 - DNA, 1476 bp, Artificial Sequence
  Description of Artificial Sequence: Synthetic polynucleotide
atgcttcttttggtgacttcccttttgctgtgcgagttgccacaccccgccttcctgcttattccccaggtacagcttcaacagagtgggccgggactggtgaaacactcccaaacactttctctgacgtgcgctatatcaggtgactctgtttcatctaattctgctgcgtggaactggattcgacaatctcccagtcgcgggttggaatggctgggacgaacatattatcggtctaagtggtataacgattatgctgtatctgttaaatctcgaattacgattaatcctgacacctccaagaaccagttctccctccagttgaactcagtcacaccggaagacactgcggtctactattgcgctcaagaagtcgagccacatgatgcattcgacatctggggccagggaacgatggtcaccgtcagcagtggcggcggcggatctgggggtggcggttctggcggtggaggatcagacatacaaatgacgcagagtccctcaagtgtgtacgcgagtgtgggggataaggtaactattacgtgcagagcgtcacaggatgttagtggatggcttgcctggtatcagcagaagccaggccttgctccacagctccttatcagtggtgcttctacacttcagggcgaggttccgagtagattctctggttctggatctggtactgacttcactcttacaatttcttctttgcaaccagaagactttgcgacttattactgccaacaggccaaatacttcccttatacatttggccaaggtaccaagttggagataaaggcggccgcaactaccacccctgcccctcggccgccgactccggccccaaccatcgcaagccaacccctctccttgcgccccgaagcttgccgcccggccgcgggtggagccgtgcatacccgggggctggactttgcctgcgatatctacatttgggccccgctggccggcacttgcggcgtgctcctgctgtcgctggtcatcaccctttactgcaagaggggccggaagaagctgctttacatcttcaagcagccgttcatgcggcccgtgcagacgactcaggaagaggacggatgctcgtgcagattccctgaggaggaagaggggggatgcgaactgcgcgtcaagttctcacggtccgccgacgcccccgcatatcaacagggccagaatcagctctacaacgagctgaacctgggaaggagagaggagtacgacgtgctggacaagcgacgcggacgcgacccggagatgggggggaaaccacggcggaaaaaccctcaggaaggactgtacaacgaactccagaaagacaagatggcggaagcctactcagaaatcgggatgaagggagagcggaggaggggaaagggtcacgacgggctgtaccagggactgagcaccgccactaaggatacctacgatgccttgcatatgcaagcactcccaccccgg

SEQ ID NO: 114 - protein, 492 aa, Artificial Sequence
  Description of Artificial Sequence: Synthetic polypeptide
MLLLVTSLLLCELPHPAFLLIPQVQLQQSGPGLVKHSQTLSLTCAISGDSVSSNSAAWNWIRQSPSRGLEWLGRTYYRSKWYNDYAVSVKSRITINPDTSKNQFSLQLNSVTPEDTAVYYCAQEVEPHDAFDIWGQGTMVTVSSGGGGSGGGGSGGGGSDIQMTQSPSSVYASVGDKVTITCRASQDVSGWLAWYQQKPGLAPQLLISGASTLQGEVPSRFSGSGSGTDFTLTISSLQPEDFATYYCQQAKYFPYTFGQGTKLEIKAAATTTPAPRPPTPAPTIASQPLSLRPEACRPAAGGAVHTRGLDFACDIYIWAPLAGTCGVLLLSLVITLYCKRGRKKLLYIFKQPFMRPVQTTQEEDGCSCRFPEEEEGGCELRVKFSRSADAPAYQQGQNQLYNELNLGRREEYDVLDKRRGRDPEMGGKPRRKNPQEGLYNELQKDKMAEAYSEIGMKGERRRGKGHDGLYQGLSTATKDTYDALHMQALPPR

SEQ ID NO: 115 - protein, 6 aa, Artificial Sequence
  Description of Artificial Sequence: Synthetic peptide
QDVSGW

SEQ ID NO: 116 - protein, 3 aa, Artificial Sequence
  Description of Artificial Sequence: Synthetic peptide
GAS

SEQ ID NO: 117 - protein, 9 aa, Artificial Sequence
  Description of Artificial Sequence: Synthetic peptide
QQAKYFPYT

SEQ ID NO: 118 - protein, 10 aa, Artificial Sequence
  Description of Artificial Sequence: Synthetic peptide
GDSVSSNSAA

SEQ ID NO: 119 - protein, 9 aa, Artificial Sequence
  Description of Artificial Sequence: Synthetic peptide
TYYRSKWYN

SEQ ID NO: 120 - protein, 12 aa, Artificial Sequence
  Description of Artificial Sequence: Synthetic peptide
AQEVEPHDAFDI

SEQ ID NO: 121 - DNA, 732 bp, Artificial Sequence
  Description of Artificial Sequence: Synthetic polynucleotide
caagtacaacttcaacagtctgggcctgggcttgtaaaacctagccaaactctgtccctcacgtgcgcgatttcaggggacagtgtaagttccaactcagccgcatggaactggatcaggcagtcaccttcaagggggctcgaatggcttggccgaacgtactacaggagtaagtggtacaacgattatgcagtgtctgtgaaatcacggattactatcaatcccgacacgtccaagaaccagttctctctgcaactcaactcagtgacaccagaggatacggccgtttactattgtgcacaggaagtgcaacctgatgatgcctttgacatttggggtcagggcacgatggttacggtaagctctgggggaggcggcagtggagggggaggtagtgggggagggggatctgatatacagatgacacaaagcccgtcatccgtcagtgcttcagttggtgataaagtaaccattacgtgccgcgcttcccaagacgttagcggatggttggcttggtatcaacaaaaaccggggttggctccgcaactcctcatatccggtgcgagtacgctccaaggcgaagtccctagcagattttccgggagcggttccggtacagatttcacgttgaccattagctctctccagcccgaagattttgcaacctactattgccaacaggccaaaaattttccatatacatttggtcaaggcactaagctcgaaatcaaa

SEQ ID NO: 122 - protein, 244 aa, Artificial Sequence
  Description of Artificial Sequence: Synthetic polypeptide
QVQLQQSGPGLVKPSQTLSLTCAISGDSVSSNSAAWNWIRQSPSRGLEWLGRTYYRSKWYNDYAVSVKSRITINPDTSKNQFSLQLNSVTPEDTAVYYCAQEVQPDDAFDIWGQGTMVTVSSGGGGSGGGGSGGGGSDIQMTQSPSSVSASVGDKVTITCRASQDVSGWLAWYQQKPGLAPQLLISGASTLQGEVPSRFSGSGSGTDFTLTISSLQPEDFATYYCQQAKNFPYTFGQGTKLEIK

SEQ ID NO: 123 - DNA, 1476 bp, Artificial Sequence
  Description of Artificial Sequence: Synthetic polynucleotide
atgcttcttttggtgacttcccttttgctgtgcgagttgccacaccccgccttcctgcttattccccaagtacaacttcaacagtctgggcctgggcttgtaaaacctagccaaactctgtccctcacgtgcgcgatttcaggggacagtgtaagttccaactcagccgcatggaactggatcaggcagtcaccttcaagggggctcgaatggcttggccgaacgtactacaggagtaagtggtacaacgattatgcagtgtctgtgaaatcacggattactatcaatcccgacacgtccaagaaccagttctctctgcaactcaactcagtgacaccagaggatacggccgtttactattgtgcacaggaagtgcaacctgatgatgcctttgacatttggggtcagggcacgatggttacggtaagctctgggggaggcggcagtggagggggaggtagtgggggagggggatctgatatacagatgacacaaagcccgtcatccgtcagtgcttcagttggtgataaagtaaccattacgtgccgcgcttcccaagacgttagcggatggttggcttggtatcaacaaaaaccggggttggctccgcaactcctcatatccggtgcgagtacgctccaaggcgaagtccctagcagattttccgggagcggttccggtacagatttcacgttgaccattagctctctccagcccgaagattttgcaacctactattgccaacaggccaaaaattttccatatacatttggtcaaggcactaagctcgaaatcaaagcggccgcaactaccacccctgcccctcggccgccgactccggccccaaccatcgcaagccaacccctctccttgcgccccgaagcttgccgcccggccgcgggtggagccgtgcatacccgggggctggactttgcctgcgatatctacatttgggccccgctggccggcacttgcggcgtgctcctgctgtcgctggtcatcaccctttactgcaagaggggccggaagaagctgctttacatcttcaagcagccgttcatgcggcccgtgcagacgactcaggaagaggacggatgctcgtgcagattccctgaggaggaagaggggggatgcgaactgcgcgtcaagttctcacggtccgccgacgcccccgcatatcaacagggccagaatcagctctacaacgagctgaacctgggaaggagagaggagtacgacgtgctggacaagcgacgcggacgcgacccggagatgggggggaaaccacggcggaaaaaccctcaggaaggactgtacaacgaactccagaaagacaagatggcggaagcctactcagaaatcgggatgaagggagagcggaggaggggaaagggtcacgacgggctgtaccagggactgagcaccgccactaaggatacctacgatgccttgcatatgcaagcactcccaccccgg

SEQ ID NO: 124 - protein, 492 aa, Artificial Sequence
  Description of Artificial Sequence: Synthetic polypeptide
MLLLVTSLLLCELPHPAFLLIPQVQLQQSGPGLVKPSQTLSLTCAISGDSVSSNSAAWNWIRQSPSRGLEWLGRTYYRSKWYNDYAVSVKSRITINPDTSKNQFSLQLNSVTPEDTAVYYCAQEVQPDDAFDIWGQGTMVTVSSGGGGSGGGGSGGGGSDIQMTQSPSSVSASVGDKVTITCRASQDVSGWLAWYQQKPGLAPQLLISGASTLQGEVPSRFSGSGSGTDFTLTISSLQPEDFATYYCQQAKNFPYTFGQGTKLEIKAAATTTPAPRPPTPAPTIASQPLSLRPEACRPAAGGAVHTRGLDFACDIYIWAPLAGTCGVLLLSLVITLYCKRGRKKLLYIFKQPFMRPVQTTQEEDGCSCRFPEEEEGGCELRVKFSRSADAPAYQQGQNQLYNELNLGRREEYDVLDKRRGRDPEMGGKPRRKNPQEGLYNELQKDKMAEAYSEIGMKGERRRGKGHDGLYQGLSTATKDTYDALHMQALPPR

SEQ ID NO: 125 - protein, 6 aa, Artificial Sequence
  Description of Artificial Sequence: Synthetic peptide
QDVSGW

SEQ ID NO: 126 - protein, 3 aa, Artificial Sequence
  Description of Artificial Sequence: Synthetic peptide
GAS

SEQ ID NO: 127 - protein, 9 aa, Artificial Sequence
  Description of Artificial Sequence: Synthetic peptide
QQAKNFPYT

SEQ ID NO: 128 - protein, 10 aa, Artificial Sequence
  Description of Artificial Sequence: Synthetic peptide
GDSVSSNSAA

SEQ ID NO: 129 - protein, 9 aa, Artificial Sequence
  Description of Artificial Sequence: Synthetic peptide
TYYRSKWYN

SEQ ID NO: 130 - protein, 12 aa, Artificial Sequence
  Description of Artificial Sequence: Synthetic peptide
AQEVQPDDAFDI

SEQ ID NO: 131 - DNA, 732 bp, Artificial Sequence
  Description of Artificial Sequence: Synthetic polynucleotide
caggtacagctgcagcagtcaggtccaggactggtgaagccctcgcagaccctctcactcacctgtgacatctccggggacagtgtctctagcaacagtgctgcttggaactggatcaggcagtccccatcgagaggccttgagtggctgggaaggacatactacaggtccaagtggtataatgattatgcagtatctgtgaaaagtcgaataaccatcaacccagacacatccaagaaccagttctccctgcagctgaactctgtgactcccgaggacacggctgtgtattactgtgcccaagagatagaacctcatgatgcttttgatatctgggaccaagggacaatggtcaccgtctcttcaggaggtggcgggtctggcggtggaggtagcggtggtggcggatccgtcatccagatgacccagtctccatcttccgtgtctgcatctgtaggagacaaagtcaccatcacttgtcgggcgagtcaggatgttagcggctggttagcctggtatcagcagaaaccagggctagcccctcagctcctgatctctggtgcatcctctttgcaaggtggagtcccatcaaggttcagcggcagtggatctgggacagattttactctcaccatcagcagcctgcagcctgaagattttgccacttattattgtcaacaggctaaatatttcccttacacttttggccaggggaccaagctggaaatcaaa

SEQ ID NO: 132 - protein, 244 aa, Artificial Sequence
  Description of Artificial Sequence: Synthetic polypeptide
QVQLQQSGPGLVKPSQTLSLTCDISGDSVSSNSAAWNWIRQSPSRGLEWLGRTYYRSKWYNDYAVSVKSRITINPDTSKNQFSLQLNSVTPEDTAVYYCAQEIEPHDAFDIWDQGTMVTVSSGGGGSGGGGSGGGGSVIQMTQSPSSVSASVGDKVTITCRASQDVSGWLAWYQQKPGLAPQLLISGASSLQGGVPSRFSGSGSGTDFTLTISSLQPEDFATYYCQQAKYFPYTFGQGTKLEIK

SEQ ID NO: 133 - DNA, 1476 bp, Artificial Sequence
  Description of Artificial Sequence: Synthetic polynucleotide
atgttgctgctcgtgacctcgctccttctgtgcgagctgccccatccggcttttctgctcatccctcaagtgcagctgcagcagtccggtcctggactggtcaagccgtcccagactctgagcctgacttgcgatattagcggggactcagtctcgtccaattcggcggcctggaactggatccggcagtcaccatcaaggggcctggaatggctcgggcgcacttactaccggtccaaatggtataacgactacgccgtgtccgtgaagtcccggatcaccattaaccccgacacctcgaagaaccagttctcactccaactgaacagcgtgacccccgaggataccgcggtgtactactgcgcacaagaaatcgaaccgcacgacgccttcgacatttgggaccagggaacgatggtcacagtgtcgtccggtggaggaggttccggaggcggtggatctggaggcggaggttcggtgatccagatgacccagagcccctcctcggtgtccgcatccgtgggcgataaggtcaccattacctgtagagcgtcccaggacgtgtccggatggctggcctggtaccagcagaagccaggcttggctcctcaactgctgatctccggcgccagctcacttcaggggggggtgccatcacgcttctccggatccggttccggcaccgacttcaccctgaccatcagcagcctccagcctgaggacttcgccacttactactgccaacaggccaagtacttcccctataccttcggacaaggcactaagctggaaatcaaggcggccgcaactaccacccctgcccctcggccgccgactccggccccaaccatcgcaagccaacccctctccttgcgccccgaagcttgccgcccggccgcgggtggagccgtgcatacccgggggctggactttgcctgcgatatctacatttgggccccgctggccggcacttgcggcgtgctcctgctgtcgctggtcatcaccctttactgcaagaggggccggaagaagctgctttacatcttcaagcagccgttcatgcggcccgtgcagacgactcaggaagaggacggatgctcgtgcagattccctgaggaggaagaggggggatgcgaactgcgcgtcaagttctcacggtccgccgacgcccccgcatatcaacagggccagaatcagctctacaacgagctgaacctgggaaggagagaggagtacgacgtgctggacaagcgacgcggacgcgacccggagatgggggggaaaccacggcggaaaaaccctcaggaaggactgtacaacgaactccagaaagacaagatggcggaagcctactcagaaatcgggatgaagggagagcggaggaggggaaagggtcacgacgggctgtaccagggactgagcaccgccactaaggatacctacgatgccttgcatatgcaagcactcccaccccgg

SEQ ID NO: 134 - protein, 492 aa, Artificial Sequence
  Description of Artificial Sequence: Synthetic polypeptide
MLLLVTSLLLCELPHPAFLLIPQVQLQQSGPGLVKPSQTLSLTCDISGDSVSSNSAAWNWIRQSPSRGLEWLGRTYYRSKWYNDYAVSVKSRITINPDTSKNQFSLQLNSVTPEDTAVYYCAQEIEPHDAFDIWDQGTMVTVSSGGGGSGGGGSGGGGSVIQMTQSPSSVSASVGDKVTITCRASQDVSGWLAWYQQKPGLAPQLLISGASSLQGGVPSRFSGSGSGTDFTLTISSLQPEDFATYYCQQAKYFPYTFGQGTKLEIKAAATTTPAPRPPTPAPTIASQPLSLRPEACRPAAGGAVHTRGLDFACDIYIWAPLAGTCGVLLLSLVITLYCKRGRKKLLYIFKQPFMRPVQTTQEEDGCSCRFPEEEEGGCELRVKFSRSADAPAYQQGQNQLYNELNLGRREEYDVLDKRRGRDPEMGGKPRRKNPQEGLYNELQKDKMAEAYSEIGMKGERRRGKGHDGLYQGLSTATKDTYDALHMQALPPR

SEQ ID NO: 135 - protein, 6 aa, Artificial Sequence
  Description of Artificial Sequence: Synthetic peptide
QDVSGW

SEQ ID NO: 136 - protein, 3 aa, Artificial Sequence
  Description of Artificial Sequence: Synthetic peptide
GAS

SEQ ID NO: 137 - protein, 9 aa, Artificial Sequence
  Description of Artificial Sequence: Synthetic peptide
QQAKYFPYT

SEQ ID NO: 138 - protein, 10 aa, Artificial Sequence
  Description of Artificial Sequence: Synthetic peptide
GDSVSSNSAA

SEQ ID NO: 139 - protein, 9 aa, Artificial Sequence
  Description of Artificial Sequence: Synthetic peptide
TYYRSKWYN

SEQ ID NO: 140 - protein, 12 aa, Artificial Sequence
  Description of Artificial Sequence: Synthetic peptide
AQEIEPHDAFDI

SEQ ID NO: 141 - DNA, 732 bp, Artificial Sequence
  Description of Artificial Sequence: Synthetic polynucleotide
caagtgcagctgcagcagtccggtcctggactggtcaagcactcccagactctgagcctggcctgcgcgattagcggggactcagtctcgtccaattcggcggcctggaactggatccggcagtcaccatcaaggggcctggaatggctcgggcgcacttactaccggtccaaatggtataacgactacgccgtgtccgtgaagtcccggatcaccattaaccccgacacctcgaagaaccagttctcactccaactgaacagcgtgacccccgaggataccgcggtgtactactgcgcacaagaagtgcagccgcaggacgccctggacatttgggggcagggaacgatggtcacagtgtcgtccggtggaggaggttccggaggcggtggatctggaggcggaggttcggatatccagatgacccagagcccctccttcgtgtccgcatccgtgggcgataaggtcattattacctgtagagcgtcccaggacgtgtccggatggctggcctggtaccagcagaagccaggcttggctcctcaactgctgatctccggcgccagcactcttcagggggaagtgccatcacgcttctccggatccggttccggcaccgacttcaccctgaccatcagcagcctccagcctgaggacttcgccacttactactgccaacaggccaagtacttcccctataccttcggacaaggcactaagctggaaatcaag

SEQ ID NO: 142 - protein, 244 aa, Artificial Sequence
  Description of Artificial Sequence: Synthetic polypeptide
QVQLQQSGPGLVKHSQTLSLACAISGDSVSSNSAAWNWIRQSPSRGLEWLGRTYYRSKWYNDYAVSVKSRITINPDTSKNQFSLQLNSVTPEDTAVYYCAQEVQPQDALDIWGQGTMVTVSSGGGGSGGGGSGGGGSDIQMTQSPSFVSASVGDKVIITCRASQDVSGWLAWYQQKPGLAPQLLISGASTLQGEVPSRFSGSGSGTDFTLTISSLQPEDFATYYCQQAKYFPYTFGQGTKLEIK

SEQ ID NO: 143 - DNA, 1476 bp, Artificial Sequence
  Description of Artificial Sequence: Synthetic polynucleotide
atgttgctgctcgtgacctcgctccttctgtgcgagctgccccatccggcttttctgctcatccctcaagtgcagctgcagcagtccggtcctggactggtcaagcactcccagactctgagcctggcctgcgcgattagcggggactcagtctcgtccaattcggcggcctggaactggatccggcagtcaccatcaaggggcctggaatggctcgggcgcacttactaccggtccaaatggtataacgactacgccgtgtccgtgaagtcccggatcaccattaaccccgacacctcgaagaaccagttctcactccaactgaacagcgtgacccccgaggataccgcggtgtactactgcgcacaagaagtgcagccgcaggacgccctggacatttgggggcagggaacgatggtcacagtgtcgtccggtggaggaggttccggaggcggtggatctggaggcggaggttcggatatccagatgacccagagcccctccttcgtgtccgcatccgtgggcgataaggtcattattacctgtagagcgtcccaggacgtgtccggatggctggcctggtaccagcagaagccaggcttggctcctcaactgctgatctccggcgccagcactcttcagggggaagtgccatcacgcttctccggatccggttccggcaccgacttcaccctgaccatcagcagcctccagcctgaggacttcgccacttactactgccaacaggccaagtacttcccctataccttcggacaaggcactaagctggaaatcaaggcggccgcaactaccacccctgcccctcggccgccgactccggccccaaccatcgcaagccaacccctctccttgcgccccgaagcttgccgcccggccgcgggtggagccgtgcatacccgggggctggactttgcctgcgatatctacatttgggccccgctggccggcacttgcggcgtgctcctgctgtcgctggtcatcaccctttactgcaagaggggccggaagaagctgctttacatcttcaagcagccgttcatgcggcccgtgcagacgactcaggaagaggacggatgctcgtgcagattccctgaggaggaagaggggggatgcgaactgcgcgtcaagttctcacggtccgccgacgcccccgcatatcaacagggccagaatcagctctacaacgagctgaacctgggaaggagagaggagtacgacgtgctggacaagcgacgcggacgcgacccggagatgggggggaaaccacggcggaaaaaccctcaggaaggactgtacaacgaactccagaaagacaagatggcggaagcctactcagaaatcgggatgaagggagagcggaggaggggaaagggtcacgacgggctgtaccagggactgagcaccgccactaaggatacctacgatgccttgcatatgcaagcactcccaccccgg

SEQ ID NO: 144 - protein, 492 aa, Artificial Sequence
  Description of Artificial Sequence: Synthetic polypeptide
MLLLVTSLLLCELPHPAFLLIPQVQLQQSGPGLVKHSQTLSLACAISGDSVSSNSAAWNWIRQSPSRGLEWLGRTYYRSKWYNDYAVSVKSRITINPDTSKNQFSLQLNSVTPEDTAVYYCAQEVQPQDALDIWGQGTMVTVSSGGGGSGGGGSGGGGSDIQMTQSPSFVSASVGDKVIITCRASQDVSGWLAWYQQKPGLAPQLLISGASTLQGEVPSRFSGSGSGTDFTLTISSLQPEDFATYYCQQAKYFPYTFGQGTKLEIKAAATTTPAPRPPTPAPTIASQPLSLRPEACRPAAGGAVHTRGLDFACDIYIWAPLAGTCGVLLLSLVITLYCKRGRKKLLYIFKQPFMRPVQTTQEEDGCSCRFPEEEEGGCELRVKFSRSADAPAYQQGQNQLYNELNLGRREEYDVLDKRRGRDPEMGGKPRRKNPQEGLYNELQKDKMAEAYSEIGMKGERRRGKGHDGLYQGLSTATKDTYDALHMQALPPR

SEQ ID NO: 145 - protein, 6 aa, Artificial Sequence
  Description of Artificial Sequence: Synthetic peptide
QDVSGW

SEQ ID NO: 146 - protein, 3 aa, Artificial Sequence
  Description of Artificial Sequence: Synthetic peptide
GAS

SEQ ID NO: 147 - protein, 9 aa, Artificial Sequence
  Description of Artificial Sequence: Synthetic peptide
QQAKYFPYT

SEQ ID NO: 148 - protein, 10 aa, Artificial Sequence
  Description of Artificial Sequence: Synthetic peptide
GDSVSSNSAA

SEQ ID NO: 149 - protein, 9 aa, Artificial Sequence
  Description of Artificial Sequence: Synthetic peptide
TYYRSKWYN

SEQ ID NO: 150 - protein, 12 aa, Artificial Sequence
  Description of Artificial Sequence: Synthetic peptide
AQEVQPQDALDI

SEQ ID NO: 151 - DNA, 732 bp, Artificial Sequence
  Description of Artificial Sequence: Synthetic polynucleotide
caggtacagctgcagcagtcaggtccaggactggtgaagccctcgcagaccctctcactcacctgtgccatctccggggacagtgtctctagcaacagtgctgcttggaactggatcaggcagtccccatcgagaggccttgagtggctgggaaggacatactacaggtccaagtggtatactgattatgcagtatctgtgaaaaatcgaataaccatcaacccagacacatccaagaatcagttctccctgcagctgaactctgtgactcccgaggacacggctgtgtattactgtgcccaagaggtagaacctcaggatgcttttgatatctggggccaagggacaatggtcaccgtctcttcaggaggtggcgggtctggcggtggaggtagcggtggtggcggatccgacatccagatgacccagtctccatcttccgtgtctgcatctgtaggagacaaagtcaccatcacttgtcgggcgagtcaggatgttagcggctggttagcctggtatcagcagaaaccagggctagcccctcagctcctgatctttggtgcatccactttgcaaggtgaagtcccatcaaggttcagcggcagtggatctgggacagattttactctcaccatcagtagcctgcagcctgaagattttgccacttattattgtcaacaggctaaatatttcccttacacttttggccgggggaccaagctggaaatcaaa

SEQ ID NO: 152 - protein, 244 aa, Artificial Sequence
  Description of Artificial Sequence: Synthetic polypeptide
QVQLQQSGPGLVKPSQTLSLTCAISGDSVSSNSAAWNWIRQSPSRGLEWLGRTYYRSKWYTDYAVSVKNRITINPDTSKNQFSLQLNSVTPEDTAVYYCAQEVEPQDAFDIWGQGTMVTVSSGGGGSGGGGSGGGGSDIQMTQSPSSVSASVGDKVTITCRASQDVSGWLAWYQQKPGLAPQLLIFGASTLQGEVPSRFSGSGSGTDFTLTISSLQPEDFATYYCQQAKYFPYTFGRGTKLEIK

SEQ ID NO: 153 - DNA, 1476 bp, Artificial Sequence
  Description of Artificial Sequence: Synthetic polynucleotide
atgttgctgctcgtgacctcgctccttctgtgcgagctgccccatccggcttttctgctcatccctcaagtgcagctgcagcagtccggtcctggactggtcaagccgtcccagactctgagcctgacttgcgcaattagcggggactcagtctcgtccaattcggcggcctggaactggatccggcagtcaccatcaaggggcctggaatggctcgggcgcacttactaccggtccaaatggtataccgactacgccgtgtccgtgaagaatcggatcaccattaaccccgacacctcgaagaaccagttctcactccaactgaacagcgtgacccccgaggataccgcggtgtactactgcgcacaagaagtggaaccgcaggacgccttcgacatttggggacagggaacgatggtcacagtgtcgtccggtggaggaggttccggaggcggtggatctggaggcggaggttcggatatccagatgacccagagcccctcctcggtgtccgcatccgtgggcgataaggtcaccattacctgtagagcgtcccaggacgtgtccggatggctggcctggtaccagcagaagccaggcttggctcctcaactgctgatcttcggcgccagcactcttcagggggaagtgccatcacgcttctccggatccggttccggcaccgacttcaccctgaccatcagcagcctccagcctgaggacttcgccacttactactgccaacaggccaagtacttcccctataccttcggaagaggcactaagctggaaatcaaggcggccgcaactaccacccctgcccctcggccgccgactccggccccaaccatcgcaagccaacccctctccttgcgccccgaagcttgccgcccggccgcgggtggagccgtgcatacccgggggctggactttgcctgcgatatctacatttgggccccgctggccggcacttgcggcgtgctcctgctgtcgctggtcatcaccctttactgcaagaggggccggaagaagctgctttacatcttcaagcagccgttcatgcggcccgtgcagacgactcaggaagaggacggatgctcgtgcagattccctgaggaggaagaggggggatgcgaactgcgcgtcaagttctcacggtccgccgacgcccccgcatatcaacagggccagaatcagctctacaacgagctgaacctgggaaggagagaggagtacgacgtgctggacaagcgacgcggacgcgacccggagatgggggggaaaccacggcggaaaaaccctcaggaaggactgtacaacgaactccagaaagacaagatggcggaagcctactcagaaatcgggatgaagggagagcggaggaggggaaagggtcacgacgggctgtaccagggactgagcaccgccactaaggatacctacgatgccttgcatatgcaagcactcccaccccgg

SEQ ID NO: 154 - protein, 492 aa, Artificial Sequence
  Description of Artificial Sequence: Synthetic polypeptide
MLLLVTSLLLCELPHPAFLLIPQVQLQQSGPGLVKPSQTLSLTCAISGDSVSSNSAAWNWIRQSPSRGLEWLGRTYYRSKWYTDYAVSVKNRITINPDTSKNQFSLQLNSVTPEDTAVYYCAQEVEPQDAFDIWGQGTMVTVSSGGGGSGGGGSGGGGSDIQMTQSPSSVSASVGDKVTITCRASQDVSGWLAWYQQKPGLAPQLLIFGASTLQGEVPSRFSGSGSGTDFTLTISSLQPEDFATYYCQQAKYFPYTFGRGTKLEIKAAATTTPAPRPPTPAPTIASQPLSLRPEACRPAAGGAVHTRGLDFACDIYIWAPLAGTCGVLLLSLVITLYCKRGRKKLLYIFKQPFMRPVQTTQEEDGCSCRFPEEEEGGCELRVKFSRSADAPAYQQGQNQLYNELNLGRREEYDVLDKRRGRDPEMGGKPRRKNPQEGLYNELQKDKMAEAYSEIGMKGERRRGKGHDGLYQGLSTATKDTYDALHMQALPPR

SEQ ID NO: 155 - protein, 6 aa, Artificial Sequence
  Description of Artificial Sequence: Synthetic peptide
QDVSGW

SEQ ID NO: 156 - protein, 3 aa, Artificial Sequence
  Description of Artificial Sequence: Synthetic peptide
GAS

SEQ ID NO: 157 - protein, 9 aa, Artificial Sequence
  Description of Artificial Sequence: Synthetic peptide
QQAKYFPYT

SEQ ID NO: 158 - protein, 10 aa, Artificial Sequence
  Description of Artificial Sequence: Synthetic peptide
GDSVSSNSAA

SEQ ID NO: 159 - protein, 9 aa, Artificial Sequence
  Description of Artificial Sequence: Synthetic peptide
TYYRSKWYT

SEQ ID NO: 160 - protein, 12 aa, Artificial Sequence
  Description of Artificial Sequence: Synthetic peptide
AQEVEPQDAFDI

SEQ ID NO: 161 - DNA, 732 bp, Artificial Sequence
  Description of Artificial Sequence: Synthetic polynucleotide
caggtacagctgcagcagtcaggtccaggactggtgaagccctcgcagaccctctcactcacctgtgccatctcagggaacagtgtctctagcaacagtgctgcttggaactggatcaggcagtccccatcgagaggccttgagtggctgggaaggacatactacaggtccaagtggtataatgattatgcagtatctgtgaaaagtcgaataaccatcaacccagacacatccaagaaccagttctccctgcagctgaactctgtgactcccgaggacacggctgtgtattactgtgcccaagaggtagaacctcaagatgcttttgatatctggggccaagggacaatggtcaccgtctcttcaggaggtggcgggtctggcggtggaggtagcggtggtggcggatccgacatccagatgacccagtctccatcttccgtgtctgcatctgtaggagacaaagtcaccatcacttgtcgggcgagtcaggatgttagcggctggttagcctggtatcagcagaaaccagggctagcccctcagctcctgatctttggtgcatccactttgcaaggtgaagtcccatcaagattcagcggcggtggatctgggacagattttactctcaccatcagcagcctgcagcctgaagattttgccacttattattgtcaacaggctaaatatttcccttacacttttggccaggggaccaagctggaaatcaaa

SEQ ID NO: 162 - protein, 244 aa, Artificial Sequence
  Description of Artificial Sequence: Synthetic polypeptide
QVQLQQSGPGLVKPSQTLSLTCAISGNSVSSNSAAWNWIRQSPSRGLEWLGRTYYRSKWYNDYAVSVKSRITINPDTSKNQFSLQLNSVTPEDTAVYYCAQEVEPQDAFDIWGQGTMVTVSSGGGGSGGGGSGGGGSDIQMTQSPSSVSASVGDKVTITCRASQDVSGWLAWYQQKPGLAPQLLIFGASTLQGEVPSRFSGGGSGTDFTLTISSLQPEDFATYYCQQAKYFPYTFGQGTKLEIK

SEQ ID NO: 163 - DNA, 1476 bp, Artificial Sequence
  Description of Artificial Sequence: Synthetic polynucleotide
atgttgctgctcgtgacctcgctccttctgtgcgagctgccccatccggcttttctgctcatccctcaagtgcagctgcagcagtccggtcctggactggtcaagccgtcccagactctgagcctgacttgcgccattagcgggaactcagtctcgtccaattcggcggcctggaactggatccggcagtcaccatcaaggggcctggaatggctcgggcgcacttactaccggtccaaatggtataacgactacgccgtgtccgtgaagtcccggatcaccattaaccccgacacctcgaagaaccagttctcactccaactgaacagcgtgacccccgaggataccgcggtgtactactgcgcacaagaagtggaaccgcaggacgccttcgacatttggggacagggaacgatggtcacagtgtcgtccggtggaggaggttccggaggcggtggatctggaggcggaggttcggatatccagatgacccagagcccctcctcggtgtccgcatccgtgggcgataaggtcaccattacctgtagagcgtcccaggacgtgtccggatggctggcctggtaccagcagaagccaggcttggctcctcaactgctgatctttggcgccagcactcttcagggggaggtgccatcacgcttctccggaggtggttccggcaccgacttcaccctgaccatcagcagcctccagcctgaggacttcgccacttactactgccaacaggccaagtacttcccctataccttcggacaaggcactaagctggaaatcaaggcggccgcaactaccacccctgcccctcggccgccgactccggccccaaccatcgcaagccaacccctctccttgcgccccgaagcttgccgcccggccgcgggtggagccgtgcatacccgggggctggactttgcctgcgatatctacatttgggccccgctggccggcacttgcggcgtgctcctgctgtcgctggtcatcaccctttactgcaagaggggccggaagaagctgctttacatcttcaagcagccgttcatgcggcccgtgcagacgactcaggaagaggacggatgctcgtgcagattccctgaggaggaagaggggggatgcgaactgcgcgtcaagttctcacggtccgccgacgcccccgcatatcaacagggccagaatcagctctacaacgagctgaacctgggaaggagagaggagtacgacgtgctggacaagcgacgcggacgcgacccggagatgggggggaaaccacggcggaaaaaccctcaggaaggactgtacaacgaactccagaaagacaagatggcggaagcctactcagaaatcgggatgaagggagagcggaggaggggaaagggtcacgacgggctgtaccagggactgagcaccgccactaaggatacctacgatgccttgcatatgcaagcactcccaccccgg

SEQ ID NO: 164 - protein, 492 aa, Artificial Sequence
  Description of Artificial Sequence: Synthetic polypeptide
MLLLVTSLLLCELPHPAFLLIPQVQLQQSGPGLVKPSQTLSLTCAISGNSVSSNSAAWNWIRQSPSRGLEWLGRTYYRSKWYNDYAVSVKSRITINPDTSKNQFSLQLNSVTPEDTAVYYCAQEVEPQDAFDIWGQGTMVTVSSGGGGSGGGGSGGGGSDIQMTQSPSSVSASVGDKVTITCRASQDVSGWLAWYQQKPGLAPQLLIFGASTLQGEVPSRFSGGGSGTDFTLTISSLQPEDFATYYCQQAKYFPYTFGQGTKLEIKAAATTTPAPRPPTPAPTIASQPLSLRPEACRPAAGGAVHTRGLDFACDIYIWAPLAGTCGVLLLSLVITLYCKRGRKKLLYIFKQPFMRPVQTTQEEDGCSCRFPEEEEGGCELRVKFSRSADAPAYQQGQNQLYNELNLGRREEYDVLDKRRGRDPEMGGKPRRKNPQEGLYNELQKDKMAEAYSEIGMKGERRRGKGHDGLYQGLSTATKDTYDALHMQALPPR

SEQ ID NO: 165 - protein, 6 aa, Artificial Sequence
  Description of Artificial Sequence: Synthetic peptide
QDVSGW

SEQ ID NO: 166 - protein, 3 aa, Artificial Sequence
  Description of Artificial Sequence: Synthetic peptide
GAS

SEQ ID NO: 167 - protein, 9 aa, Artificial Sequence
  Description of Artificial Sequence: Synthetic peptide
QQAKYFPYT

SEQ ID NO: 168 - protein, 10 aa, Artificial Sequence
  Description of Artificial Sequence: Synthetic peptide
GNSVSSNSAA

SEQ ID NO: 169 - protein, 9 aa, Artificial Sequence
  Description of Artificial Sequence: Synthetic peptide
TYYRSKWYN

SEQ ID NO: 170 - protein, 12 aa, Artificial Sequence
  Description of Artificial Sequence: Synthetic peptide
AQEVEPQDAFDI

SEQ ID NO: 171 - DNA, 732 bp, Artificial Sequence
  Description of Artificial Sequence: Synthetic polynucleotide
caggtacagctgcagcagtcaggtccaggactggtgaagccctcgcagaccctctcactcacctgtgccatctccggggacagtgtctctagcaacagtgctgcttggaactggatcaggcagtccccatcgagaggccttgagtggctgggaaggacatactacaggtccaagtggtataatgattatgcagtatctgtgaaaagtcgaataaccatcaacccagacacatccaagaaccagttctccctgcagctgaactctgtgactcccgaggacacggctgtgtattactgtgcccaagaggtagaacctcatgatgctcttgatatctggggccaagggacaatggtcaccgtctcttcaggaggtggcgggtctggcggtggaggtagcggtggtggcggatccgacatccagatgacgcagtctccatcatccgtgtctgcatctgtaggagacaaagtcaccatcacttgtcgggcgagtcaggatgttagcggctggttagcctggtatcaacagaaaccagggctagcccctcagctcctgatctttggtgcatccactttgcaaggtgaagtcccatcaaggttcagcggcagtggatctgggacagattttactctcaccatcagcagcctgcagcctgaagattttgccacttattattgtcaacaggctaaatatttcccttacacttttggccaggggaccaagctggagatcaaa

SEQ ID NO: 172 - protein, 244 aa, Artificial Sequence; identical to SEQ ID NO: 72
  Description of Artificial Sequence: Synthetic polypeptide

SEQ ID NO: 173 - DNA, 1476 bp, Artificial Sequence
  Description of Artificial Sequence: Synthetic polynucleotide
atgttgctgctcgtgacctcgctccttctgtgcgagctgccccatccggcttttctgctcatccctcaagtgcagctgcagcagtccggtcctggactggtcaagccgtcccagactctgagcctgacttgcgcgattagcggggactcagtctcgtccaattcggcggcctggaactggatccggcagtcaccatcaaggggcctggaatggctcgggcgcacttactaccggtccaaatggtataacgactacgccgtgtccgtgaagtcccggatcaccattaaccccgacacctcgaagaaccagttctcactccaactgaacagcgtgacccccgaggataccgcggtgtactactgcgcacaagaagtggaaccgcacgacgccctggacatttggggtcagggaacgatggtcacagtgtcgtccggtggaggaggttccggaggcggtggatctggaggcggaggttcggatatccagatgacccagagcccctcctcggtgtccgcatccgtgggcgataaggtcaccattacctgtagagcgtcccaggacgtgtccggatggctggcctggtaccagcagaagccaggcttggctcctcaactgctgatcttcggcgccagcacacttcagggggaggtgccatcacgcttctccggatccggttccggcaccgacttcaccctgaccatcagcagcctccagcctgaggacttcgccacttactactgccaacaggccaagtacttcccctataccttcggacaaggcactaagctggaaatcaaggcggccgcaactaccacccctgcccctcggccgccgactccggccccaaccatcgcaagccaacccctctccttgcgccccgaagcttgccgcccggccgcgggtggagccgtgcatacccgggggctggactttgcctgcgatatctacatttgggccccgctggccggcacttgcggcgtgctcctgctgtcgctggtcatcaccctttactgcaagaggggccggaagaagctgctttacatcttcaagcagccgttcatgcggcccgtgcagacgactcaggaagaggacggatgctcgtgcagattccctgaggaggaagaggggggatgcgaactgcgcgtcaagttctcacggtccgccgacgcccccgcatatcaacagggccagaatcagctctacaacgagctgaacctgggaaggagagaggagtacgacgtgctggacaagcgacgcggacgcgacccggagatgggggggaaaccacggcggaaaaaccctcaggaaggactgtacaacgaactccagaaagacaagatggcggaagcctactcagaaatcgggatgaagggagagcggaggaggggaaagggtcacgacgggctgtaccagggactgagcaccgccactaaggatacctacgatgccttgcatatgcaagcactcccaccccgg

SEQ ID NO: 174 - protein, 492 aa, Artificial Sequence; identical to SEQ ID NO: 74
  Description of Artificial Sequence: Synthetic polypeptide

SEQ ID NO: 175 - protein, 6 aa, Artificial Sequence
  Description of Artificial Sequence: Synthetic peptide
QDVSGW

SEQ ID NO: 176 - protein, 3 aa, Artificial Sequence
  Description of Artificial Sequence: Synthetic peptide
GAS

SEQ ID NO: 177 - protein, 9 aa, Artificial Sequence
  Description of Artificial Sequence: Synthetic peptide
QQAKYFPYT

SEQ ID NO: 178 - protein, 10 aa, Artificial Sequence
  Description of Artificial Sequence: Synthetic peptide
GDSVSSNSAA

SEQ ID NO: 179 - protein, 9 aa, Artificial Sequence
  Description of Artificial Sequence: Synthetic peptide
TYYRSKWYN

SEQ ID NO: 180 - protein, 12 aa, Artificial Sequence
  Description of Artificial Sequence: Synthetic peptide
AQEVEPHDALDI

SEQ ID NO: 181 - DNA, 66 bp, Artificial Sequence
  Description of Artificial Sequence: Synthetic oligonucleotide
atttgggccccgctggccggcacttgcggcgtgctcctgctgtcgctggtcatcaccctttactgc

SEQ ID NO: 182 - protein, 22 aa, Artificial Sequence
  Description of Artificial Sequence: Synthetic peptide
IWAPLAGTCGVLLLSLVITLYC

SEQ ID NO: 183 - DNA, 141 bp, Artificial Sequence
  Description of Artificial Sequence: Synthetic polynucleotide
actaccacccctgcccctcggccgccgactccggccccaaccatcgcaagccaacccctctccttgcgccccgaagcttgccgcccggccgcgggtggagccgtgcatacccgggggctggactttgcctgcgatatctac

SEQ ID NO: 184 - protein, 47 aa, Artificial Sequence
  Description of Artificial Sequence: Synthetic polypeptide
TTTPAPRPPTPAPTIASQPLSLRPEACRPAAGGAVHTRGLDFACDIY

SEQ ID NO: 185 - protein, 69 aa, Artificial Sequence
  Description of Artificial Sequence: Synthetic polypeptide
TTTPAPRPPTPAPTIASQPLSLRPEACRPAAGGAVHTRGLDFACDIYIWAPLAGTCGVLLLSLVITLYC

SEQ ID NO: 186 - DNA, 126 bp, Artificial Sequence
  Description of Artificial Sequence: Synthetic polynucleotide
aagaggggccggaagaagctgctttacatcttcaagcagccgttcatgcggcccgtgcagacgactcaggaagaggacggatgctcgtgcagattccctgaggaggaagaggggggatgcgaactg

SEQ ID NO: 187 - protein, 42 aa, Artificial Sequence
  Description of Artificial Sequence: Synthetic polypeptide
KRGRKKLLYIFKQPFMRPVQTTQEEDGCSCRFPEEEEGGCEL

SEQ ID NO: 188 - DNA, 336 bp, Artificial Sequence
  Description of Artificial Sequence: Synthetic polynucleotide
cgcgtcaagttctcacggtccgccgacgcccccgcatatcaacagggccagaatcagctctacaacgagctgaacctgggaaggagagaggagtacgacgtgctggacaagcgacgcggacgcgacccggagatgggggggaaaccacggcggaaaaaccctcaggaaggactgtacaacgaactccagaaagacaagatggcggaagcctactcagaaatcgggatgaagggagagcggaggaggggaaagggtcacgacgggctgtaccagggactgagcaccgccactaaggatacctacgatgccttgcatatgcaagcactcccaccccgg

SEQ ID NO: 189 - protein, 112 aa, Artificial Sequence
  Description of Artificial Sequence: Synthetic polypeptide
RVKFSRSADAPAYQQGQNQLYNELNLGRREEYDVLDKRRGRDPEMGGKPRRKNPQEGLYNELQKDKMAEAYSEIGMKGERRRGKGHDGLYQGLSTATKDTYDALHMQALPPR

SEQ ID NO: 190 - DNA, 66 bp, Artificial Sequence
  Description of Artificial Sequence: Synthetic oligonucleotide
atgctgctgctggtgaccagcctgctgctgtgcgaactgccgcatccggcgtttctgctgattccg

SEQ ID NO: 191 - protein, 22 aa, Artificial Sequence
  Description of Artificial Sequence: Synthetic peptide
MLLLVTSLLLCELPHPAFLLIP

SEQ ID NO: 192 - DNA, 726 bp, Artificial Sequence
  Description of Artificial Sequence: Synthetic polynucleotide
gacattcagatgactcagaccacctcttccttgtccgcgtcactgggagacagagtgaccatctcgtgtcgcgcaagccaggatatctccaagtacctgaactggtaccaacagaagcccgacgggactgtgaagctgctgatctaccacacctcacgcctgcacagcggagtgccaagcagattctccggctccggctcgggaaccgattactcgcttaccattagcaacctcgagcaggaggacatcgctacctacttctgccagcaaggaaataccctgccctacaccttcggcggaggaaccaaattggaaatcaccggcggaggaggctccgggggaggaggttccgggggcgggggttccgaagtgaagctccaggagtccggccccggcctggtggcgccgtcgcaatcactctctgtgacctgtaccgtgtcgggagtgtccctgcctgattacggcgtgagctggattcggcagccgccgcggaagggcctggaatggctgggtgtcatctggggatccgagactacctactacaactcggccctgaagtcccgcctgactatcatcaaagacaactcgaagtcccaggtctttctgaagatgaactccctgcaaactgacgacaccgccatctattactgtgctaagcactactactacggtggaagctatgctatggactactgggggcaaggcacttcggtgactgtgtcaagc

SEQ ID NO: 193 - protein, 242 aa, Artificial Sequence
  Description of Artificial Sequence: Synthetic polypeptide
DIQMTQTTSSLSASLGDRVTISCRASQDISKYLNWYQQKPDGTVKLLIYHTSRLHSGVPSRFSGSGSGTDYSLTISNLEQEDIATYFCQQGNTLPYTFGGGTKLEITGGGGSGGGGSGGGGSEVKLQESGPGLVAPSQSLSVTCTVSGVSLPDYGVSWIRQPPRKGLEWLGVIWGSETTYYNSALKSRLTIIKDNSKSQVFLKMNSLQTDDTAIYYCAKHYYYGGSYAMDYWGQGTSVTVSS

SEQ ID NO: 194 - DNA, 1470 bp, Artificial Sequence
  Description of Artificial Sequence: Synthetic polynucleotide
atgcttctcctggtcacctccctgctcctctgcgaactgcctcaccctgccttccttctgattcctgacattcagatgactcagaccacctcttccttgtccgcgtcactgggagacagagtgaccatctcgtgtcgcgcaagccaggatatctccaagtacctgaactggtaccaacagaagcccgacgggactgtgaagctgctgatctaccacacctcacgcctgcacagcggagtgccaagcagattctccggctccggctcgggaaccgattactcgcttaccattagcaacctcgagcaggaggacatcgctacctacttctgccagcaaggaaataccctgccctacaccttcggcggaggaaccaaattggaaatcaccggcggaggaggctccgggggaggaggttccgggggcgggggttccgaagtgaagctccaggagtccggccccggcctggtggcgccgtcgcaatcactctctgtgacctgtaccgtgtcgggagtgtccctgcctgattacggcgtgagctggattcggcagccgccgcggaagggcctggaatggctgggtgtcatctggggatccgagactacctactacaactcggccctgaagtcccgcctgactatcatcaaagacaactcgaagtcccaggtctttctgaagatgaactccctgcaaactgacgacaccgccatctattactgtgctaagcactactactacggtggaagctatgctatggactactgggggcaaggcacttcggtgactgtgtcaagcgcggccgcaactaccacccctgcccctcggccgccgactccggccccaaccatcgcaagccaacccctctccttgcgccccgaagcttgccgcccggccgcgggtggagccgtgcatacccgggggctggactttgcctgcgatatctacatttgggccccgctggccggcacttgcggcgtgctcctgctgtcgctggtcatcaccctttactgcaagaggggccggaagaagctgctttacatcttcaagcagccgttcatgcggcccgtgcagacgactcaggaagaggacggatgctcgtgcagattccctgaggaggaagaggggggatgcgaactgcgcgtcaagttctcacggtccgccgacgcccccgcatatcaacagggccagaatcagctctacaacgagctgaacctgggaaggagagaggagtacgacgtgctggacaagcgacgcggacgcgacccggagatgggggggaaaccacggcggaaaaaccctcaggaaggactgtacaacgaactccagaaagacaagatggcggaagcctactcagaaatcgggatgaagggagagcggaggaggggaaagggtcacgacgggctgtaccagggactgagcaccgccactaaggatacctacgatgccttgcatatgcaagcactcccaccccgg

SEQ ID NO: 195 - protein, 490 aa, Artificial Sequence
  Description of Artificial Sequence: Synthetic polypeptide
MLLLVTSLLLCELPHPAFLLIPDIQMTQTTSSLSASLGDRVTISCRASQDISKYLNWYQQKPDGTVKLLIYHTSRLHSGVPSRFSGSGSGTDYSLTISNLEQEDIATYFCQQGNTLPYTFGGGTKLEITGGGGSGGGGSGGGGSEVKLQESGPGLVAPSQSLSVTCTVSGVSLPDYGVSWIRQPPRKGLEWLGVIWGSETTYYNSALKSRLTIIKDNSKSQVFLKMNSLQTDDTAIYYCAKHYYYGGSYAMDYWGQGTSVTVSSAAATTTPAPRPPTPAPTIASQPLSLRPEACRPAAGGAVHTRGLDFACDIYIWAPLAGTCGVLLLSLVITLYCKRGRKKLLYIFKQPFMRPVQTTQEEDGCSCRFPEEEEGGCELRVKFSRSADAPAYQQGQNQLYNELNLGRREEYDVLDKRRGRDPEMGGKPRRKNPQEGLYNELQKDKMAEAYSEIGMKGERRRGKGHDGLYQGLSTATKDTYDALHMQALPPR

SEQ ID NO: 196 - DNA, 1482 bp, Artificial Sequence
  Description of Artificial Sequence: Synthetic polynucleotide
atgcttcttttggtgacttcccttttgctgtgcgagttgccacaccccgccttcctgcttattccccaggtacagctccagcagagtggcccagggctcgtgaagccaagccagacgctgtccctgacttgtgcaatttcaggggattcagtttcatcaaatagcgcggcgtggaattggattcgacaatctccttcccgagggttggaatggcttggacgaacatattacagatccaaatggtataacgactatgcggtatcagtaaagtcaagaataaccattaaccccgacacaagcaagaaccaattctctttgcagcttaactctgtcacgccagaagacacggcagtctattattgcgctcgcgaggtaacgggtgacctggaagacgcttttgacatttgggggcagggtacgatggtgacagtcagttcagggggcggtgggagtgggggagggggtagcggggggggagggtcagacattcagatgacccagtccccttcatccttgtctgcctccgtcggtgacagggtgacaataacatgcagagcaagccaaacaatctggagctatctcaactggtaccagcagcgaccaggaaaagcgccaaacctgctgatttacgctgcttcctccctccaatcaggcgtgcctagtagatttagcggtaggggctccggcaccgattttacgctcactataagctctcttcaagcagaagattttgcgacttattactgccagcagtcctatagtatacctcagactttcggacagggtaccaagttggagattaaggcggccgcaactaccacccctgcccctcggccgccgactccggccccaaccatcgcaagccaacccctctccttgcgccccgaagcttgccgcccggccgcgggtggagccgtgcatacccgggggctggactttgcctgcgatatctacatttgggccccgctggccggcacttgcggcgtgctcctgctgtcgctggtcatcaccctttactgcaagaggggccggaagaagctgctttacatcttcaagcagccgttcatgcggcccgtgcagacgactcaggaagaggacggatgctcgtgcagattccctgaggaggaagaggggggatgcgaactgcgcgtcaagttctcacggtccgccgacgcccccgcatatcaacagggccagaatcagctctacaacgagctgaacctgggaaggagagaggagtacgacgtgctggacaagcgacgcggacgcgacccggagatgggggggaaaccacggcggaaaaaccctcaggaaggactgtacaacgaactccagaaagacaagatggcggaagcctactcagaaatcgggatgaagggagagcggaggaggggaaagggtcacgacgggctgtaccagggactgagcaccgccactaaggatacctacgatgccttgcatatgcaagcactcccaccccgg

SEQ ID NO: 197 - protein, 494 aa, Artificial Sequence
  Description of Artificial Sequence: Synthetic polypeptide
MLLLVTSLLLCELPHPAFLLIPQVQLQQSGPGLVKPSQTLSLTCAISGDSVSSNSAAWNWIRQSPSRGLEWLGRTYYRSKWYNDYAVSVKSRITINPDTSKNQFSLQLNSVTPEDTAVYYCAREVTGDLEDAFDIWGQGTMVTVSSGGGGSGGGGSGGGGSDIQMTQSPSSLSASVGDRVTITCRASQTIWSYLNWYQQRPGKAPNLLIYAASSLQSGVPSRFSGRGSGTDFTLTISSLQAEDFATYYCQQSYSIPQTFGQGTKLEIKAAATTTPAPRPPTPAPTIASQPLSLRPEACRPAAGGAVHTRGLDFACDIYIWAPLAGTCGVLLLSLVITLYCKRGRKKLLYIFKQPFMRPVQTTQEEDGCSCRFPEEEEGGCELRVKFSRSADAPAYQQGQNQLYNELNLGRREEYDVLDKRRGRDPEMGGKPRRKNPQEGLYNELQKDKMAEAYSEIGMKGERRRGKGHDGLYQGLSTATKDTYDALHMQALPPR

SEQ ID NO: 198 - DNA, 732 bp, Artificial Sequence
  Description of Artificial Sequence: Synthetic polynucleotide
gaggtccagctggtacagtctgggggaggcttggtacagcctggggggtccctgagactctcctgtgcagcctctggattcacctttgatgattatgccatgcactgggtccggcaagctccagggaagggcctggagtgggtctcaggtattagttggaatagtggtagcataggctatgcggactctgtgaagggccgattcaccatctccagagacaacgccaagaactccctgtatctgcaaatgaacagtctgagagctgaggacacggccttgtattactgtgcaaaagatttatcgtcagtggctggaccctttaactactggggccagggcaccctggtcaccgtctcctcaggaggtggcgggtctggtggaggcggtagcggcggtggcggatcctcttctgagctgactcaggaccctgctgtgtctgtggccttgggacagacagtcaggatcacatgccaaggagacagcctcagaagctattatgcaagctggtaccagcagaagccaggacaggcccctgtacttgtcatctatggtaaaaacaaccggccctcagggatcccagaccgattctctggctccagctcaggaaacacagcttccttgaccatcactggggctcaggcggaggatgaggctgactattactgtaactcccgggacagcagtggtaaccatctggtattcggcggaggcacccagctgaccgtcctcggt

SEQ ID NO: 199 - protein, 244 aa, Artificial Sequence
  Description of Artificial Sequence: Synthetic polypeptide
EVQLVQSGGGLVQPGGSLRLSCAASGFTFDDYAMHWVRQAPGKGLEWVSGISWNSGSIGYADSVKGRFTISRDNAKNSLYLQMNSLRAEDTALYYCAKDLSSVAGPFNYWGQGTLVTVSSGGGGSGGGGSGGGGSSSELTQDPAVSVALGQTVRITCQGDSLRSYYASWYQQKPGQAPVLVIYGKNNRPSGIPDRFSGSSSGNTASLTITGAQAEDEADYYCNSRDSSGNHLVFGGGTQLTVLG

SEQ ID NO: 200 - DNA, 1476 bp, Artificial Sequence
  Description of Artificial Sequence: Synthetic polynucleotide
atgctgctgctggtgaccagcctgctgctgtgcgaactgccgcatccggcgtttctgctgattccggaggtccagctggtacagtctgggggaggcttggtacagcctggggggtccctgagactctcctgtgcagcctctggattcacctttgatgattatgccatgcactgggtccggcaagctccagggaagggcctggagtgggtctcaggtattagttggaatagtggtagcataggctatgcggactctgtgaagggccgattcaccatctccagagacaacgccaagaactccctgtatctgcaaatgaacagtctgagagctgaggacacggccttgtattactgtgcaaaagatttatcgtcagtggctggaccctttaactactggggccagggcaccctggtcaccgtctcctcaggaggtggcgggtctggtggaggcggtagcggcggtggcggatcctcttctgagctgactcaggaccctgctgtgtctgtggccttgggacagacagtcaggatcacatgccaaggagacagcctcagaagctattatgcaagctggtaccagcagaagccaggacaggcccctgtacttgtcatctatggtaaaaacaaccggccctcagggatcccagaccgattctctggctccagctcaggaaacacagcttccttgaccatcactggggctcaggcggaggatgaggctgactattactgtaactcccgggacagcagtggtaaccatctggtattcggcggaggcacccagctgaccgtcctcggtgcggccgcaactaccacccctgcccctcggccgccgactccggccccaaccatcgcaagccaacccctctccttgcgccccgaagcttgccgcccggccgcgggtggagccgtgcatacccgggggctggactttgcctgcgatatctacatttgggccccgctggccggcacttgcggcgtgctcctgctgtcgctggtcatcaccctttactgcaagaggggccggaagaagctgctttacatcttcaagcagccgttcatgcggcccgtgcagacgactcaggaagaggacggatgctcgtgcagattccctgaggaggaagaggggggatgcgaactgcgcgtcaagttctcacggtccgccgacgcccccgcatatcaacagggccagaatcagctctacaacgagctgaacctgggaaggagagaggagtacgacgtgctggacaagcgacgcggacgcgacccggagatgggggggaaaccacggcggaaaaaccctcaggaaggactgtacaacgaactccagaaagacaagatggcggaagcctactcagaaatcgggatgaagggagagcggaggaggggaaagggtcacgacgggctgtaccagggactgagcaccgccactaaggatacctacgatgccttgcatatgcaagcactcccaccccgg

SEQ ID NO: 201 - protein, 492 aa, Artificial Sequence
  Description of Artificial Sequence: Synthetic polypeptide
MLLLVTSLLLCELPHPAFLLIPEVQLVQSGGGLVQPGGSLRLSCAASGFTFDDYAMHWVRQAPGKGLEWVSGISWNSGSIGYADSVKGRFTISRDNAKNSLYLQMNSLRAEDTALYYCAKDLSSVAGPFNYWGQGTLVTVSSGGGGSGGGGSGGGGSSSELTQDPAVSVALGQTVRITCQGDSLRSYYASWYQQKPGQAPVLVIYGKNNRPSGIPDRFSGSSSGNTASLTITGAQAEDEADYYCNSRDSSGNHLVFGGGTQLTVLGAAATTTPAPRPPTPAPTIASQPLSLRPEACRPAAGGAVHTRGLDFACDIYIWAPLAGTCGVLLLSLVITLYCKRGRKKLLYIFKQPFMRPVQTTQEEDGCSCRFPEEEEGGCELRVKFSRSADAPAYQQGQNQLYNELNLGRREEYDVLDKRRGRDPEMGGKPRRKNPQEGLYNELQKDKMAEAYSEIGMKGERRRGKGHDGLYQGLSTATKDTYDALHMQALPPR

SEQ ID NO: 202 - DNA, 339 bp, Artificial Sequence
  Description of Artificial Sequence: Synthetic polynucleotide
gaggtgcagctggtggagtctgggggaggcttggtacagcctggagggtccctgagactctcctgtgcagcctctggattcaccttcagtagctatggcatgagctgggtccgccaggctccaagacaagggcttgagtgggtggccaacataaagcaagatggaagtgagaaatactatgcggactcagtgaagggccgattcaccatctccagagacaattccaagaacacgctgtatctgcaaatgaacagcctgagagccgaggacacagccacgtattactgtgcgaaagaaaatgtggactggggccagggcaccctggtcaccgtctcctca

SEQ ID NO: 203 - protein, 113 aa, Artificial Sequence
  Description of Artificial Sequence: Synthetic polypeptide
EVQLVESGGGLVQPGGSLRLSCAASGFTFSSYGMSWVRQAPRQGLEWVANIKQDGSEKYYADSVKGRFTISRDNSKNTLYLQMNSLRAEDTATYYCAKENVDWGQGTLVTVSS

SEQ ID NO: 204 - DNA, 1083 bp, Artificial Sequence
  Description of Artificial Sequence: Synthetic polynucleotide
atgctgctgctggtgaccagcctgctgctgtgcgaactgccgcatccggcgtttctgctgattccggaggtgcagctggtggagtctgggggaggcttggtacagcctggagggtccctgagactctcctgtgcagcctctggattcaccttcagtagctatggcatgagctgggtccgccaggctccaagacaagggcttgagtgggtggccaacataaagcaagatggaagtgagaaatactatgcggactcagtgaagggccgattcaccatctccagagacaattccaagaacacgctgtatctgcaaatgaacagcctgagagccgaggacacagccacgtattactgtgcgaaagaaaatgtggactggggccagggcaccctggtcaccgtctcctcagcggccgcaactaccacccctgcccctcggccgccgactccggccccaaccatcgcaagccaacccctctccttgcgccccgaagcttgccgcccggccgcgggtggagccgtgcatacccgggggctggactttgcctgcgatatctacatttgggccccgctggccggcacttgcggcgtgctcctgctgtcgctggtcatcaccctttactgcaagaggggccggaagaagctgctttacatcttcaagcagccgttcatgcggcccgtgcagacgactcaggaagaggacggatgctcgtgcagattccctgaggaggaagaggggggatgcgaactgcgcgtcaagttctcacggtccgccgacgcccccgcatatcaacagggccagaatcagctctacaacgagctgaacctgggaaggagagaggagtacgacgtgctggacaagcgacgcggacgcgacccggagatgggggggaaaccacggcggaaaaaccctcaggaaggactgtacaacgaactccagaaagacaagatggcggaagcctactcagaaatcgggatgaagggagagcggaggaggggaaagggtcacgacgggctgtaccagggactgagcaccgccactaaggatacctacgatgccttgcatatgcaagcactcccaccccgg

SEQ ID NO: 205 - protein, 361 aa, Artificial Sequence
  Description of Artificial Sequence: Synthetic polypeptide
MLLLVTSLLLCELPHPAFLLIPEVQLVESGGGLVQPGGSLRLSCAASGFTFSSYGMSWVRQAPRQGLEWVANIKQDGSEKYYADSVKGRFTISRDNSKNTLYLQMNSLRAEDTATYYCAKENVDWGQGTLVTVSSAAATTTPAPRPPTPAPTIASQPLSLRPEACRPAAGGAVHTRGLDFACDIYIWAPLAGTCGVLLLSLVITLYCKRGRKKLLYIFKQPFMRPVQTTQEEDGCSCRFPEEEEGGCELRVKFSRSADAPAYQQGQNQLYNELNLGRREEYDVLDKRRGRDPEMGGKPRRKNPQEGLYNELQKDKMAEAYSEIGMKGERRRGKGHDGLYQGLSTATKDTYDALHMQALPPR

SEQ ID NO: 206 - protein, 4 aa, Artificial Sequence
  Description of Artificial Sequence: Synthetic peptide
GFLG